European Patent Application EP 4 269 432 A1, published November 1, 2023. Title: Production of therapeutic antibodies by the microalgae Phaeodactylum tricornutum. Applicant: UNIVERSITE DE ROUEN NORMANDIE. The sequence listing filed with the application follows.

SEQUENCE LISTING (91 sequences)

SEQ ID NO: 1 - protein, 19 aa, artificial
  Signal peptide E of azurocidine
MTRLTVLALLAGLLASSRA

SEQ ID NO: 2 - protein, 19 aa, artificial
  Signal peptide H5
MDWTWRFLFVVAAATGVQS

SEQ ID NO: 3 - protein, 19 aa, artificial
  Signal peptide H7
MEFGLSWVFLVALFRGVQC

SEQ ID NO: 4 - protein, 22 aa, artificial
  Signal peptide L1
MDMRVPAQLLGLLLLWLSGARC

SEQ ID NO: 5 - protein, 18 aa, artificial
  Signal peptide B
MKWVTFISLLFLFSSAYS

SEQ ID NO: 6 - protein, 17 aa, artificial
  Signal peptide of the human BIP protein
MKLSLVAAMLLLLSAAR

SEQ ID NO: 7 - protein, 20 aa, artificial
  Signal peptide of the BIP protein from Phaeodactylum tricornutum
MMFMRIAVAALALLAAPSIR

SEQ ID NO: 8 - protein, 20 aa, artificial
  Signal peptide of the BIP protein from Phaeodactylum tricornutum
MIFMRIAVAALALLAAPSIR

SEQ ID NO: 9 - protein, 16 aa, artificial
  Signal peptide of the human PDI protein
MLRRALLCLAVAALVR

SEQ ID NO: 10 - protein, 20 aa, artificial
  Self-cleaving linker peptide E2A
QCTNYALLKLAGDVESNPGP

SEQ ID NO: 11 - protein, 22 aa, artificial
  Self-cleaving linker peptide F2A
VKQTLNFDLLKLAGDVESNPGP

SEQ ID NO: 12 - protein, 27 aa, artificial
  Self-cleaving linker peptide variant of F2A
KIVAPVKQTLNFDLLKLAGDVESNPGP

SEQ ID NO: 13 - protein, 24 aa, artificial
  Self-cleaving linker peptide variant of F2A
APVKQTLNFDLLKLAGDVESNPGP

SEQ ID NO: 14 - protein, 19 aa, artificial
  Self-cleaving linker peptide P2A
ATNFSLLKQAGDVEENPGP

SEQ ID NO: 15 - protein, 18 aa, artificial
  Self-cleaving linker peptide T2A
EGRGSLLTCGDVEENPGP

SEQ ID NO: 16 - DNA, 23 bp, artificial
  wild type encephalomyocarditis virus (EMCV) internal ribosomal entry site (IRES)
atgataatatggccacaaccatg

SEQ ID NO: 17 - DNA, 46 bp, artificial
  mutated EMCV IRES with attenuated translation efficiency (IRESatt)
atgataagcttgccacaaccccgggagatgaggatcgtttcgcatg

SEQ ID NO: 18 - protein, 4 aa, artificial
  furin-cleavage site
RRKR

SEQ ID NO: 19 - DNA, 241 bp, artificial
  Termination sequence of the FcpA gene
accttccttaaaaatttaattttcattagttgcagtcactccgctttggtttcacagtcaggaataacactagctcgtcttcaccatggatgccaatctcgcctattcatggtgtataaaagttcaacatccaaagctagaacttttggaaagagaaagaatatccgaatagggcacggcgtgccgtattgttggagtggactagcagaaagtgaggaaggcacaggatgagttttctcga

SEQ ID NO: 20 - DNA, 273 bp, artificial
  Termination sequence of the NR gene
caatttactttaagactagcgcaatttttttcttacattagatgaacataaaacgacgatgaggatcactgttagggaaacgatgaactacgctgaggacttcctattattcgtcctttgatggcgtggttgttctttggtttgcggccgagcgcaacgaccaaggcctgtaccaaaaacgaagttgataatcagatatttgagttgtaacaagaaactaaagcattattttagcagtagcacgaatcaggatctaaaatgaacgcatccgga

SEQ ID NO: 21 - DNA, 501 bp, artificial
  Termination sequence of the H4-1B gene
gcttgcgcttgatcctcgactttgttgctcgtctttaaaaccttggaacgattatatacaatcaccaactcaaaaaccggattttctaaaatccacccaaacaaccaaagaaaatacttctcattgcatttatgaatcacagcagacctgcgtccttttaaaacttagatcctgttttcttataaaaaacagatcaaattttctgggagttcattgactctgccagtcagaatcaatcctgcagtaattctttatttacaggtgaaagtaaaagagaatcccaattttttgcttgtacattaaggtcctccttacattacagctaatttcaaaataagatgaagttggattcgtgtcctttcatggtgatgtgatattctgcactataccaaacaccgtgaaatgtcagctagagcttgtcatgaggcagttgctgccaatcactacatatagatccttcacggagaaaagttggcttcattctctgttgctaatcggctg

SEQ ID NO: 22 - DNA, 501 bp, artificial
  Termination sequence of the V-ATPase C gene
acggacgtttgttggagattccgcttttacctgatttccagttcctgtaattttgtcgttccttatgtttccacacaaacgactgcaagcaaaatcaactaatttgtttatcacatttcaatagccagtttgaatgtttttcttacgatactgtaggcagtggaagcggaattggtttttgtgggcaaccgaaaaaggcttgcaattttcaattagggtaacagtagtcggtaaacaattgctcatctagctctaggaagtctattaatccacaggttggaaacgcaatgaatgtgccatgtatgacggcgccggtgtaggcaggagaatttctctaatgtaatctttgttccacgactcttacagaggcacccaaaccatcgcttcgatcagttgacgagaggtttctgaaaacgatcttatcgaggcgccgttggtggtcctttcgaaagaatcacttccaacatgtagctttgggatgcaaaactttcattggatgtg

SEQ ID NO: 23 - DNA, 501 bp, artificial
  Termination sequence of the gamma-tubulin gene
agcaaactcattatgatgcatgggagtgcgaccgagtttcgaacgatgctaacgaacattattagtggaaggcagtcattgttgtatgcgtcaaagtatataatcagacggacagtagttcattttaaacttttgttcggaaagcgttgatcattcatcggggaatcgcgctaacgagcagtaattggagttgtaactgcaggctcaacgcgtttctggctcccgtgggttaccataatgctaactatcattctttatttgcagtatcaccagtccaagaattattcgtggtcatttctgatgctactgtggagaagtgagagtaatttcgccgactttgaagtgaagacgcgtctccgaacgtagattgttggtattgtaccattgaaggagagtttttgaactcaggttgttgatcgtaatgtccgcgacatcctggcgcactacacgccaatgaccataacatgtcttggtcgccctcctcgtaagtcatcgccattg

SEQ ID NO: 24 - DNA, 598 bp, artificial
  promoter of the H4-1B gene
gtctctttcccgggaaacgggtacactcctccgcgccaacaacatattactactactaccaagaacgtccacggccttgtcgtgcgttacgctctcccaacgcgtgcggggtaaattacgtctcggtttgctaagtagcgcacagctaaatagatgaccgttattgtatttaagatcattcaatattgattgcattgtactttgcgtcaaactgaaattccctcgtactaacggttaacccgtcaaccctaagcgttcgcccaaagtagtcaaccgggacacgcgaaccgacattgggcagatctttcacagacagaaaaccatttccaatccaaataagcatgactattacacacccattcgtagcgcgaggacaaactgatagctccaacaaaatgcgccaacatcgtacattgtaagaagcttacggaacactatgtatgtagaaccatacgaacagcaactagtactggccatcgagcagcggtgactcccggctttcgtagcgctgtgaaggttacactctcacaattcgctctcggctacaaccgacaaaagtcttactcacagtcaataccgaaaacaaacaacagccaac

SEQ ID NO: 25 - DNA, 500 bp, artificial
  promoter of the V-ATPase C gene
cgattggaatggttttggagaggaaaccgtttttatggcggttggatgggaaaggaagggatggtgttcacactcagatttgggagctcacccaccgtatgttgacagtacaaacaatcctgcaatcctgcgaaccaactgtttctcgtctttttggtctgtacgtggtaggatagagagtctgccgggataccatttcgtgcgcagacgtggaagagtcattattcagcttgcacgacacagattttatacagacaaacgtacaatacgcaattgctccgacaaaaattgccgaccattcctacaggcatatttttgcatataattaggggaaacgcatagaatgcaatcttcagttacatacagacaacattctgtcgcagctcgccacacgtaccaactccagattccgagcttcgccgcggccttttggaaagatcgaaaaggcgccgccgcggctgtcgttcccgcagaaagtgcaagcagccactagcgcaaaa

SEQ ID NO: 26 - DNA, 422 bp, artificial
  promoter of the NR gene of Phaeodactylum tricornutum
catatgcggaagtgactgtaaacgagaagtgcacgaagccttttcttgtgacgtcacaaaccgaacagccctacgtggcgtgcgactttccggcactttggatatcgttgccctatatgtattgggtgtatacatgtcgtattccaactacgacagaaaacagtcagttacgggtattcgaacttccggcacctgcagcgaggagttttgtgtccgtcgcacatcctccgtgctttcggcacctacgtaggcggcaaacttcctgccttccgcccgccttgcggcattccggctccgggccagaattgcccgggtgttcacaattttgcctcctcacgaaaaaacgttctactttgtattttggtcgggtttcggatccttccagcaaccattctcattcaaagtcaccacttgtgcgaacg

SEQ ID NO: 27 - DNA, 444 bp, artificial
  promoter of the fcpA/lhcf1 gene of Phaeodactylum tricornutum
gggctgcaggacgcaatggaggattatcaccgcaaaaatgaacttcgaaaaaaactttcgagcgaccatggaaaaggaggatcagattcagattacaacagtggattgctctggtagcaaatatcttctgctagattggctcatggtcggttttggacgttcgaagctcaccgtcaaaagaaacaaaagagaagaatgacgtcttcgtgacgtagaatctacgactgtactcggatctgggaaatgaattgactcacggtcttcttcgagtcctgttacaggcccttggtccgaacccccacacgatttttgcaccaaagatttgcttcaatttgctggatgttttgactgcaagatcagctggcctagcaagagtgctcgtgttgcttcgtcgggaatccctacgaatttcagttctgcacaaatttgtctgccgtttcgaga

SEQ ID NO: 28 - DNA, 187 bp, artificial
  promoter of the fcpb /lhcf2 gene of Phaeodactylum tricornutum
gagattcaaaattcaatctgtttggacctggataagacacaagagcgacatcctgacatgaacgccgtaaacagcaaatcctggttgaacacgtatccttttgggggcctcccgctacgacgctcgctccagctggggcttccttactatacacagcgcgcatatttcacggttgccagatgtcaag

SEQ ID NO: 29 - DNA, 1246 bp, artificial
  Promoter of the Phatr3_J37038 gene
tgtcgctacttcaccacagctttattgaatagggacgagcttttattaatcatgtgctgctgtcctttttgcatcaggattgtcacgtagccactttggactgtaattaatcttgacttctttatctaacaaagcggcgagatcaaggtccttctcagtcaaaccctgcagcttgtgtgtccaaatttttacctcgatatctcggtaactagtaagatggaagtcggggtggtgactttcgcgttcagctatggcccccatctcgttgatgcattttaaagcagactgaaaattgcgtgccgtaaatttacgagatatatgcaaaggttctgattcactcgagcaaagattccacagcgatccccttatcccaagtttgtccactgcactttcaaatgtcaatagaaaagatgcgtccagagtagagcaaggagcgcaatgtttcggtccttgcggggagcctgaagccatcactaatactgtgaaaatgagagccggcaatttctgaagactatgtaagtctccgaacaggaaggaagcgcaagcaaaccacaattcgaactccagataaacttgctgttagcacaatcaacatgaccatgtacaagcgtcgtctgcttgtgagcccgtcaatatgattgattgagggcagatccttagcactttaaccctgtaaacatttttgttttggctctcatcaacggcagctgtagcgaatctatagcctgccgggcagtataacgttcatgatcaaaaatgaagtgtatataagtcgataaatgtaaccctttttcttgctatataattttttttgaacgatgaacactaaacacacatagctatctgacatcgaacataaatgtaagagtcattccaaataagtagagatgcaatgtggacatcatgggatgatgtgtggatttacgatcccctcaactgtaaaactattcttaggcacaatttaccgagcgaacaaaaatactaaagaaacttagcatattttcgaaagcattgtaattttcaacctttgtgaaattttttctatattttccgaagtgtgacagtgaattccaaatcttgagtctgctttgtgtactttgacatgacaactttcggacacgctcactttttgacgaccacacgttcaatcgttgctgcgctccggcacagactaaagttcaggaattgcttgtcacctacgcagcatcaccactctctcgtctctaccgtgattcaaggctgaatc

SEQ ID NO: 30 - DNA, 1125 bp, artificial
  Promoter of the Phatr3_Jdraft1443 gene
tcgggttggagtactgctaggagcaccataagccaaagactatgtgctgctggtgaactctaaaagcggacggcaattaacggtttgtgtttcttaaccattgtcatgatggtggtcgtcgaggttgtttctcgtcgttgttagcaagattcaaccctgcatctcggtataaagtgcgcaatgcgtctacagcaactcaccatcaatctgcgatcttgttcgttcgcaagaccacgaaatttgctggccttcaggaaaggaaaatactgttggtctatatccgagtcttggagtagggcaacacgacaatgctgtgctgtatatgaagtcagacaacacaccacaaacccatactcccaaataaatgtatagcgatttatcgaaagagctcggttcaaagaatttgtccaaacatggtcggaaatattccaaaagcgacaaaggctaagtaagctaagtcctcttggtgcttgaaaggaaagctgcagaggggatgatttaaaattacgcgaaaggaaggagcttctaagatggagagagagagagaccgcagtcatgtttacaaagtgaagctacaaaatggccagaacaaatgatgtactattttggctacgtgtaggtggaccggtcctattggccaaatgagcccaaacagaaccctagccacaatttttttactaattaagctgtggtctttcttatgcgtcaggtgggtttcatttctcgaagaacgttttcgctccccgaggcggtcttgctccattagtcaatgatgtcacgcataccatattcctgcgactaccgtctcaaataaagccggtaacgcaacaatatgtaggctgatgttatggtgtgatttaacaaggcccaaacagttttttaacaggttactattggcgattcaagacatcacaataatgaccatcttaaacgattcagagtgtgactcatccgggaaagtagggtcgcatgtttcctgagagaatcgcttcatgagatctcatcggttgcaactggtctcacaagtgaacgttagataagcaataacagcaaacctttgtgatttcagctaactgtgaccagatcgcttctagactggaaacaactctcatccattccacgact

SEQ ID NO: 31 - DNA, 535 bp, artificial
  Promoter of the Phatr3_J35102 gene
taattatcattgtatgttcgttctctaggaatttatagtcaagcttccttttgctactaccctgctcctcaatcagcgtcagggaagcaagatcctcctcggctagggtcttagcatggttcttggcctacgctagctaggaaggtaccataaaaacgagagctattaatggctcagcatttatccgatacatgtttaacagaaagacagaaaacacgaaaaaagttgttgacagtgaatgctccagatgtcacaagaaaggcgttggggcgaatcgattgggcctttggaggcattagtaaaaaggagaaagctttttaatctttgtcgacatgtacttctatacaatattgctatagaattgaaggacagcttgaaatgtctatcgacatagtgactccgacttaaggtcattcactatttttacgcgtgaccgcggacccaaaacccgaccggcagttcctgccccaaacataatacaaattatagctccaaaattgactctctttgaaccgacgacccaattggttctacc

SEQ ID NO: 32 - DNA, 1098 bp, artificial
  Promoter of the Phatr3_J50252 gene
aaattgtatactccagcagtcgtttaataccggagacggtagacgcaagagcagctcacactctttggccacgactgtaaatgcctctagtgttgacgagtttgcgtgcacgagagaaattttcgagagaacacaggaaggaccccagtacttttgggtccttttgagcttgcaacgcttttcgtttcgaaaaccaaatccaaatccctttcgacacaggggctttttctcgcgcatgtgataaaaagcaaacaaaacccggagatcatccaaggtcgtcactgtcagaatacggtgactctagaaggcaatgcggaactcccagccggccgcatactattgacgatgaatcatcttgcttttcattactataggttgttggccgcctctcgatttattttcgagtgatctgtttaaaatgttcctcattcggtgaattttcttgcagaccatgtcccaagtcctacactaccacagcagatgatggaattaaggtcaccgtcaaaaggtagacagagtcgcgttagaaaccatgttagataaagggtcaaacggaatgttgcggattccccagggctatagacaggactaccaaagagatctgcgatcaaaattttgttgcacagcacatataccgaaagataacttgagttatccttacattgggagtcccaaaaatcaatctttcgagcgtcttcgtgccgcaacaattagatggccagttggaacaaaaaaagtatcaaatggtcgaaaatacccaagagaaacgctcactaatagaattctgtctgcctcttatatttctttgaacatgagcgttattagcaggtaaacagttgtttcgtaaatctgacattaatagtggagtgtggtcataatgccgcgctcctctgatgtcgaaactatggattcattgaaaacggtcatcggtcatagcaaaggaacttcgctttctagtaaataaccacacaaacaaatttcctcacctctttcgttgaatctggcatttccatcaacaccttttcatagctttgtggatggattgagttgcgctcgctgtcaccatttgcgccgaattccttgccctttacagtaatg

SEQ ID NO: 33 - DNA, 957 bp, artificial
  Promoter of the Phatr3_J34085 gene
aatcataggcaatgtttggtacacaataaatttgacgtagttcattatgtgctgcaatactgaatacttgccaggagtgacaggattctagctcctgaggagcgcttacagtggaattacacacatgacttgtaccgacagccaactaactataataagaagcaatgcggacttggtaggatcctttcatcaattcaaacattcactatcaatcaaaaattacaaattttacttgcttgcagtcagcatatatttgtcaacgcattgggttctttcatagtcaaatagaaatgtcacgagaatagctcccgggcccgtcaagttcttaattctgtaacttgtccttgccactccatttgcacttgacgtatcacttgtcgctctcaacacagcattacacaatggcactctacagagcattggttaatgtaaattattgaaaggcaaaacatagcccttcttgactgtgagtcccaccatcgctacgagtcacttacatgtaaaatatctgtccttccatcgagggcacggaattctgaaacgaaaacaatcttgttgggctcggtagtccgttacgcaaaaacgcttctatcaattcaattaggattggtcttggtttggagctgcccgacgcgctcaaaaattgactgggtatgggtacactttctctctgtcgaaatattttgtacagtcattttggttcttgggtatgcttattggagatgatcagttgatgcgcgacggattgagcccaaacaatttacatcatagagatatgcactttggaaaagaccctctgcggtcatctgcaaatcccacaagctttttgctctcgaaccttcacaatcttacccgagttgctatcgttgctagcagcctttcccattgattgccaacattttgatcctgacaacccatagattcgctctgttaaaccaacagcaacagcaagcaaat

SEQ ID NO: 34 - DNA, 872 bp, artificial
  Promoter of the Phatr3_J48164 gene
gttgaaactacattgttgtcggatgactcgccgactgcgatacgatagattggtgatcgggcgatcggcaatgaaagacagcccgctgcgattgcagcttggcgtgctctccgtgtggtagactagtgaagcaacgaggaagcggccaaagagcttgtgaaaggtgggcatcgaatcaaaggaatagctaattgtatttccacttcaagaagaaaagatacaactgagcgattgtcactatacttttcaagttggagagcagttgtcactggattttgtctccctactagaaccgacggtcgaagatctgactggtgcgatgtgcacgagaaaaatatcataccggttggtagtcttttgaaatgtctctttggatttgaaagcgaatcgagatttttatcacagtcaattttagtttgtttcggttagatagaactgtaaacttgaacaattgtaaataatcattgagacataagttccgtcggaaatactttaagcagtttgtgtgcaaacatgtacaaacatttacttacttatatctactgtcgcatggagattttgcgttcttgtcttttagttttgcttcccgcttatgcttcttagttcaagttgtgaaacagtgccatacttcttcagcaggatactaacataaatcgattttctttcccccttacagttaataggtcaaatggaagtagtcatcattttcatggcatcgcgctggctaccgagacatttcaggaatcggttgaagtaataaaacttgaaaacccgaataaactgctctggcatcttggcgagtttcgcaagcacttacatctcacaacagcaatactcgtttcctccgttgtgtagaaacaagcctagagaat

SEQ ID NO: 35 - DNA, 953 bp, artificial
  Promoter of the Phatr3_EG02422 gene
ttaccaccaagcgctcttctatctaccagtcaacactaatgataatgcacgtatatgaatgacatatttgtttttggactaaagattgacttgatctgtatcattaaaacttgtaggcggcgtggcattgagacacaggctgtatttcgccgcaaaaagcatgaagtctcgttttgaaggggcgggatcgtcctacacctgtactccgtcattgttgtgcacactaggatgtgaaagcttgtcgaaaggagtcatgtcaggactggacagagaaacaagcaaacctaacatgacgatgtctgactgtttggattctgaagggtgattacgttgcttggcttacattaattcatgtttttatttactgtcagtagacataaatagcgatttttcggtgaactaatttttttcaaagtgtttcgttgaaagcagtaggatcggacgcagagcatttacgggttcacatgaggtttgaaaggacgagcgttcccttgcgtctgacacaaatcatagatgtttcacctggcgcgacgatcttcctgacggaacgctaaatatggccactagattgccaacccatatgtatttcaatagtggaaaagcccgtcaagacctaggcccaagtatatattcggaaggacatgtccgatatatctctacaaaggatgagcggagtcacactcggtcgtagcgtctttcaaacacttgctctcttggtttcatttttatcggtcatttggtcattgagcaaaaaggccctctggtagcgtttgtaggcatcgctacggcaaatgcctgttcagcacggtcacgagccattcgctcttgttcgttgggccacttttctcggatttgtgaagagtttcagcatcagtcgtcaaaatatcaaattatattcagaggtcaacagcgcttctgccaaattgcaactctatcgaaaaaacagaacgaac

SEQ ID NO: 36 - DNA, 1092 bp, artificial
  Promoter of the Phatr3_J42538 gene
gaagatgagcagtttccgcatcacccgaagggacacatcattacacgagattaatctaagcaaaactcagctcaagaaaggcgatgttccaacaagcggttggtatggctcttgttgcaatgcaaaaaagctcagaaaaaactagctttccgaccttttacgtatttcttggtaattcgtagaagacgcggcgacgactcacttttaaccttttgtgactgtctcgcccatcgtctacaattagttgttgctgactgtgaccaacaaacggagactctttgcccatgtctttcgttttacgtcgcaaaatgacagtcgtgtgcttctcgggattgactgtgagtcggtgtgacagactctcgcaatcgaaaatgcttcataatacccaatagagatacggttgtactaagtcatcactctaactctgtcgcggtaaatgtgaagatgtatttcgaatgtagaattgacagtgaatgccatggattgtgcgggctaaatatttgtgttatatgcaagagttttgcgatgtaattatctaatcaaactttttcattgtaacaagagaaaaggctagagatggagctatgggccgattgtgttttgaaatcacgtacaaatacatactggttctacgtgttacgtcctcaaccccacctaaactggtactgactgtgaattcgcgcggaaatatatacgtgtagttgtgggcaccaacctatctgaatcactcctagttatccctatcagaatagtctatggtgaatttcattgaagtgaacccgagtcgatacagcaaaccctatctagaaaacggggatgataaagcaaaaagaaaaggcttatttgtaaatcgtgtagatccatcaatcggtactggtagaatcgatccaggaatgctattcaatatactatcctgtttgtcgggattgttccatcagaaatcgagtagaactggtacaggctcgaccgccagctgtttctgttcgagaaaatcttttcatcaaactgcttcctcactctgaaaaagctttggtttcattccggccacaaatctgaaaagacatctttcatcgatcccggatctcaaccacc

SEQ ID NO: 37 - DNA, 985 bp, artificial
  Promoter of the Phatr3_J48356 gene
cctttaggagaacaagctgcggaaggacagcgaataatcgaagaatgtatggggcgaggggcgcatccagtataaagtgaaatatcgatagggatggaagcacgacgaaggaaagtttaattcgctgatccagttctggatgagtccttgtctttgcggtcttccgttaagttacttactgttagtgttactgttgttcagaggcaaacttgcgtctgtccttcggagtttttttgttcgcagtcgctggctggtcgtgtccgtgttgctgtctatgtaccgcgtttggaccactgctcgtaaatgcacgcctaccagatgaggaacatttccatatagtgtctcacagtcgtgttttgaatcattcactagtatcccatcacgattgcaagcacccatgcctttcattcgtagttagtgggctgattctctacacttattgttggtagcagccgaggaagacattttctctgtgacactttcaaaggtggtttccgcaaacgactccgattgttacaattaggtcaagattaagaggttcgtacctcttatacgcgcaaagaacaagattcagaagaaaaaaatgattcttagctcgtaggttcgggcattggtctctcaagaggtctatagttattgcgtttttaataagcttctattgttcgccttagtctttagctcgtaaatgactacgtttcacattgttgcaaaaatggaaaacaacggtgtataacctagaatgtacaaatgctggatgtctccttagccgcggccactgtatcgatcgatcctttccggcagagccaaatatgttcaattcgtctatactagaattaagatggtctttgatgccttcgagctcgaatgaccaatcaaaaatcttgccggtcccctcatgaattagaacacaaatcgagggagctctcattttctctcacatatttcagtctagtaggcataattttaccaaaaggctgcagcgaag

SEQ ID NO: 38 - protein, 221 aa, artificial
  light chain of the antibody TrastuzumAb (Herceptin)
DIVMTQTPLSSPVTLGQPASISCRSSQSLVHSDGNTYLSWLQQRPGQPPRLLIYKISNRFSGVPDRFSGSGAGTDFTLKISRVEAEDVGVYYCMQATQFPHQWTFGQGTKVEIKRTVAAPSVFIFPPSDEQLKSGTASVVCLLNNFYPREAKVQWKVDNALQSGNSQESVTEQDSKDSTYSLSSTLTLSKADYEKHKVYACEVTHQGLSSPVTKSFNRGEC

SEQ ID NO: 39 - protein, 294 aa, artificial
  Heavy chain of the antibody TrastuzumAb (Herceptin)
EVHLVESGGGLVQPGGALRLSCAASGFTFSNYDMHWVRQATGKGLEWVSANGTAGDTYYPGSVKGRFTISRENAKNSLYLQMNSLRAGDTAVYYCARDVDIVATITDYFDYWGQGTLVTVSSASTKGPSVFPLAPSSKSTSGGTAALGCLVKDYFPEPVTVSWNSGALTSGVHTFPAVLQSSGLYSLSSVVTVPSSSLGTQTYICNVNHKPSNTKVDKRVEPKSCDKTHTCPPCPAPELLGGPSVFLFPPKPKDTLMISRTPEVTCVVVDVSHEDPEVKFNWYVDGVEVHNAKT

SEQ ID NO: 40 - protein, 213 aa, artificial
  light chain of the antibody RituximAb
QIVLSQSPAILSASPGEKVTMTCRASSSVSYIHWFQQKPGSSPKPWIYATSNLASGVPVRFSGSGSGTSYSLTISRVEAEDAATYYCQQWTSNPPTFGGGTKLEIKRTVAAPSVFIFPPSDEQLKSGTASVVCLLNNFYPREAKVQWKVDNALQSGNSQESVTEQDSKDSTYSLSSTLTLSKADYEKHKVYACEVTHQGLSSPVTKSFNRGEC

SEQ ID NO: 41 - protein, 451 aa, artificial
  heavy chain of the antibody RituximAb
QVQLQQPGAELVKPGASVKMSCKASGYTFTSYNMHWVKQTPGRGLEWIGAIYPGNGDTSYNQKFKGKATLTADKSSSTAYMQLSSLTSEDSAVYYCARSTYYGGDWYFNVWGAGTTVTVSAASTKGPSVFPLAPSSKSTSGGTAALGCLVKDYFPEPVTVSWNSGALTSGVHTFPAVLQSSGLYSLSSVVTVPSSSLGTQTYICNVNHKPSNTKVDKKVEPKSCDKTHTCPPCPAPELLGGPSVFLFPPKPKDTLMISRTPEVTCVVVDVSHEDPEVKFNWYVDGVEVHNAKTKPREEQYNSTYRVVSVLTVLHQDWLNGKEYKCKVSNKALPAPIEKTISKAKGQPREPQVYTLPPSRDELTKNQVSLTCLVKGFYPSDIAVEWESNGQPENNYKTTPPVLDSDGSFFLYSKLTVDKSRWQQGNVFSCSVMHEALHNHYTQKSLSLSPGK

SEQ ID NO: 42 - DNA, 5722 bp, artificial
  Nucleotide sequence of NVB5
ttcatatgcggaagtgactgtaaacgagaagtgcacgaagccttttcttgtgacgtcacaaaccgaacagccctacgtggcgtgcgactttccggcactttggatatcgttgccctatatgtattgggtgtatacatgtcgtattccaactacgacagaaaacagtcagttacgggtattcgaacttccggcacctgcagcgaggagttttgtgtccgtcgcacatcctccgtgctttcggcacctacgtaggcggcaaacttcctgccttccgcccgccttgcggcattccggctccgggccagaattgcccgggtgttcacaattttgcctcctcacgaaaaaacgttctactttgtattttggtcgggtttcggatccttccagcaaccattctcattcaaagtcaccacttgtgcgaacgatctatggatttccaagtacaaatcttcagttttctacttatctcggccagtgtaataattagtaggggcgacattgtcatgacacaaactcctctatcctcacctgtgacccttggacaacccgcctctatcagctgccgttcctcccaatcgctggtccattccgatggaaacacgtacttgtcttggctccaacagcgccctgggcagcccccgcggctcttgatttataaaataagtaacagatttagcggcgttccggaccggttcagtggttcgggcgcaggtaccgatttcacccttaagatctcccgcgtagaggccgaggatgtaggagtgtattactgtatgcaagcaactcaatttccccaccaatggacgttcggtcaagggactaaagttgaaattaagcgtacggttgctgcgccatccgtctttatttttccgccatctgacgaacagctcaaaagcggaacggcttctgtcgtctgtctcctgaacaatttttacccgcgagaggctaaggttcagtggaaggtcgataatgcgttgcagtcgggcaactcgcaggaatctgtgacggaacaggacagcaaggactccacatacagcttatcgtcgacattgacactgtcaaaagcggactacgagaaacacaaggtgtatgcctgcgaagttacccatcagggattgtcatcaccagtgaccaaatcatttaatcgaggtgaatgcgagggccgagggtcgctcttgacgtgcggtgacgtcgaagaaaacccgggacccatggattttcaggtccaaatattttcttttcttctgatatcagcctctgtcattataagtcggggggaagtccacctcgtggaaagcggggggggtttagtacagccgggtggcgccttgagactctcttgtgcagcctcgggattcaccttttcaaactacgatatgcattgggtgaggcaggccaccggcaagggtctggagtgggtgagtgctaatggcaccgcaggtgatacttattatccaggtagcgtcaaaggccgtttcacgattagtcgcgaaaacgctaagaattctctctatttgcagatgaattcactacgagcaggtgacacagcagtctactattgtgcgagggacgttgatattgttgcgaccatcaccgattacttcgattactggggtcaaggcactttggtaacagtttctagtgcgagtactaagggtccgagtgtatttcctttagccccttcctctaaaagcacttcaggcggaacagcagcccttggctgtttggtgaaagactacttcccggaacctgtaactgtgagctggaattctggcgcgctcactagtggagttcacacttttccagccgtgttacagtcatcgggtctttattccctgtcctccgtcgtgaccgtcccgtcgagttcactaggtacgcagacatacatttgtaacgtcaatcacaagccatcgaacacaaaggtggacaagcgtgttgaacccaagagctgcgataagacccacacctgccctccctgcccagctcccgagcttctcggcggaccttcggttttcctctttccgccgaagcccaaagatactttgatgatttcacggacgccagaagtgacatgcgtggttgttgacgtaagccatgaggatccggaagtgaaatttaactggtacgtcgatggagttgaggtccataacgccaagaccaagccccgcgaggaacaatataattccacatatcgtgtggtgtcggtacttacggtccttcatcaggactggctaaatggaaaagaatacaaatgcaaggtgtccaataaagcgctccccgctcccatcgaaaagacgatcagcaaggcgaaggggcaaccacgtgaaccgcaagtatacacgctcccgccctcccgagaagaaatgacaaaaaaccaagtctccctgacctgtttggttaaaggattttacccttcggacatcgcggtagagtgggagtccaacggacaacctgagaataactacaaaacgactcctccagtcctggactcggacggatccttcttcttgtactccaaattgacggttgacaaatcccgatggcaacaaggcaacgtttttagctgctcggtcatgcatgaagctttgcacaaccactacacacaaaaatcgttgtcgctgtcgccaggaaaataaaaccaccttccttaaaaatttaattttcattagttgcagtcactccgctttggtttcacagtcaggaataacactagctcgtcttcaccatggatgccaatctcgcctattcatggtgtataaaagttcaacatccaaagctagaacttttggaaagagaaagaatatccgaatagggcacggcgtgccgtattgttggagtggactagcagaaagtgaggaaggcacaggatgagttttctcgagagcccaggcatcaaataaaacgaaaggctcagtcgaaagactgggcctttcgttttatctgttgtttgtcggtgaacgctctctactagagtcacactggctcaccttcgggtgggcctttctgcgtttatatagagggaaatgtgcgcggaacccctatttgtttatttttctaaatacattcaaatatgtatccgctcatgagacaataaccctgataaatgcttcaataatattgaaaaaggaagagtatgagtattcaacatttccgtgtcgcccttattcccttttttgcggcattttgccttcctgtttttgctcacccagaaacgctggtgaaagtaaaagatgctgaagatcagttgggtgcacgagtgggttacatcgaactggatctcaacagcggtaagatccttgagagttttcgccccgaagaacgttttccaatgatgagcacttttaaagttctgctatgtggcgcggtattatcccgtattgacgccgggcaagagcaactcggtcgccgcatacactattctcagaatgacttggttgagtactcaccagtcacagaaaagcatcttacggatggcatgacagtaagagaattatgcagtgctgccataaccatgagtgataacactgcggccaacttacttctgacaacgatcggaggaccgaaggagctaaccgcttttttgcacaacatgggggatcatgtaactcgccttgatcgttgggaaccggagctgaatgaagccataccaaacgacgagcgtgacaccacgatgcctgtagcaatggcaacaacgttgcgcaaactattaactggcgaactacttactctagcttcccggcaacaattaatagactggatggaggcggataaagttgcaggaccacttctgcgctcggcccttccggctggctggtttattgctgataaatctggagccggtgagcgtgggtcacgcggtatcattgcagcactggggccagatggtaagccctcccgtatcgtagttatctacacgacggggagtcaggcaactatggatgaacgaaatagacagatcgctgagataggtgcctcactgattaagcattggtaactgtcagaccaagtttactcatatatactttagattgatttaaaacttcatttttaatttaaaaggatctaggtgaagatcctttttgataatctcatgaccaaaatcccttaacgtgagttttcgttccactgagcgtcagaccccgtagaaaagatcaaaggatcttcttgagatcctttttttctgcgcgtaatctgctgcttgcaaacaaaaaaaccaccgctaccagcggtggtttgtttgccggatcaagagctaccaactctttttccgaaggtaactggcttcagcagagcgcagataccaaatactgttcttctagtgtagccgtagttaggccaccacttcaagaactctgtagcaccgcctacatacctcgctctgctaatcctgttaccagtggctgctgccagtggcgataagtcgtgtcttaccgggttggactcaagacgatagttaccggataaggcgcagcggtcgggctgaacggggggttcgtgcacacagcccagcttggagcgaacgacctacaccgaactgagatacctacagcgtgagctatgagaaagcgccacgcttcccgaagggagaaaggcggacaggtatccggtaagcggcagggtcggaacaggagagcgcacgagggagcttccagggggaaacgcctggtatctttatagtcctgtcgggtttcgccacctctgacttgagcgtcgatttttgtgatgctcgtcaggggggcggagcctatggaaaaacgccagcaacgcggcctttttacggttcctggccttttgctggccttttgctcacatgttctttcctgcgttatcccctgattctgtggataaccgtattaccgccagagaatataaaaagccagattattaatccggcttttttattatttgacgcgttttgagattcaaaattcaatctgtttggacctggataagacacaagagcgacatcctgacatgaacgccgtaaacagcaaatcctggttgaacacgtatccttttgggggcctcccgctacgacgctcgctccagctggggcttccttactatacacagcgcgcatatttcacggttgccagatgtcaagatggccaagttgaccagtgccgttccggtgctcaccgcgcgcgacgtcgccggagcggtcgagttctggaccgaccggctcgggttctcccgggacttcgtggaggacgacttcgccggtgtggtccgggacgacgtgaccctgttcatcagcgcggtccaggaccaggtggtgccggacaacaccctggcctgggtgtgggtgcgcggcctggacgagctgtacgccgagtggtcggaggtcgtgtccacgaacttccgggacgcctccgggccggccatgaccgagatcggcgagcagccgtgggggcgggagttcgccctgcgcgacccggccggcaactgcgtgcacttcgtggccgaggagcaggactgaaccttccttaaaaatttaattttcattagttgcagtcactccgctttggtttcacagtcaggaataacactagctcgtcttcaccatggatgccaatctcgcctattcatggtgtataaaagttcaacatccaaagctagaacttttggaaagagaaagaatatccgaatagggcacggcgtgccgtattgttggagtggactagcagaaagtgaggaaggcacaggatgagttttctcgatt

SEQ ID NO: 43 - DNA, 6157 bp, artificial
  Vector NVB6
ttgtctctttcccgggaaacgggtacactcctccgcgccaacaacatattactactactaccaagaacgtccacggccttgtcgtgcgttacgctctcccaacgcgtgcggggtaaattacgtctcggtttgctaagtagcgcacagctaaatagatgaccgttattgtatttaagatcattcaatattgattgcattgtactttgcgtcaaactgaaattccctcgtactaacggttaacccgtcaaccctaagcgttcgcccaaagtagtcaaccgggacacgcgaaccgacattgggcagatctttcacagacagaaaaccatttccaatccaaataagcatgactattacacacccattcgtagcgcgaggacaaactgatagctccaacaaaatgcgccaacatcgtacattgtaagaagcttacggaacactatgtatgtagaaccatacgaacagcaactagtactggccatcgagcagcggtgactcccggctttcgtagcgctgtgaaggttacactctcacaattcgctctcggctacaaccgacaaaagtcttactcacagtcaataccgaaaacaaacaacagccaacatctatggatttccaagtacaaatcttcagttttctacttatctcggccagtgtaataattagtaggggcgacattgtcatgacacaaactcctctatcctcacctgtgacccttggacaacccgcctctatcagctgccgttcctcccaatcgctggtccattccgatggaaacacgtacttgtcttggctccaacagcgccctgggcagcccccgcggctcttgatttataaaataagtaacagatttagcggcgttccggaccggttcagtggttcgggcgcaggtaccgatttcacccttaagatctcccgcgtagaggccgaggatgtaggagtgtattactgtatgcaagcaactcaatttccccaccaatggacgttcggtcaagggactaaagttgaaattaagcgtacggttgctgcgccatccgtctttatttttccgccatctgacgaacagctcaaaagcggaacggcttctgtcgtctgtctcctgaacaatttttacccgcgagaggctaaggttcagtggaaggtcgataatgcgttgcagtcgggcaactcgcaggaatctgtgacggaacaggacagcaaggactccacatacagcttatcgtcgacattgacactgtcaaaagcggactacgagaaacacaaggtgtatgcctgcgaagttacccatcagggattgtcatcaccagtgaccaaatcatttaatcgaggtgaatgcgagggccgagggtcgctcttgacgtgcggtgacgtcgaagaaaacccgggacccatggattttcaggtccaaatattttcttttcttctgatatcagcctctgtcattataagtcggggggaagtccacctcgtggaaagcggggggggtttagtacagccgggtggcgccttgagactctcttgtgcagcctcgggattcaccttttcaaactacgatatgcattgggtgaggcaggccaccggcaagggtctggagtgggtgagtgctaatggcaccgcaggtgatacttattatccaggtagcgtcaaaggccgtttcacgattagtcgcgaaaacgctaagaattctctctatttgcagatgaattcactacgagcaggtgacacagcagtctactattgtgcgagggacgttgatattgttgcgaccatcaccgattacttcgattactggggtcaaggcactttggtaacagtttctagtgcgagtactaagggtccgagtgtatttcctttagccccttcctctaaaagcacttcaggcggaacagcagcccttggctgtttggtgaaagactacttcccggaacctgtaactgtgagctggaattctggcgcgctcactagtggagttcacacttttccagccgtgttacagtcatcgggtctttattccctgtcctccgtcgtgaccgtcccgtcgagttcactaggtacgcagacatacatttgtaacgtcaatcacaagccatcgaacacaaaggtggacaagcgtgttgaacccaagagctgcgataagacccacacctgccctccctgcccagctcccgagcttctcggcggaccttcggttttcctctttccgccgaagcccaaagatactttgatgatttcacggacgccagaagtgacatgcgtggttgttgacgtaagccatgaggatccggaagtgaaatttaactggtacgtcgatggagttgaggtccataacgccaagaccaagccccgcgaggaacaatataattccacatatcgtgtggtgtcggtacttacggtccttcatcaggactggctaaatggaaaagaatacaaatgcaaggtgtccaataaagcgctccccgctcccatcgaaaagacgatcagcaaggcgaaggggcaaccacgtgaaccgcaagtatacacgctcccgccctcccgagaagaaatgacaaaaaaccaagtctccctgacctgtttggttaaaggattttacccttcggacatcgcggtagagtgggagtccaacggacaacctgagaataactacaaaacgactcctccagtcctggactcggacggatccttcttcttgtactccaaattgacggttgacaaatcccgatggcaacaaggcaacgtttttagctgctcggtcatgcatgaagctttgcacaaccactacacacaaaaatcgttgtcgctgtcgccaggaaaataaaaccgcttgcgcttgatcctcgactttgttgctcgtctttaaaaccttggaacgattatatacaatcaccaactcaaaaaccggattttctaaaatccacccaaacaaccaaagaaaatacttctcattgcatttatgaatcacagcagacctgcgtccttttaaaacttagatcctgttttcttataaaaaacagatcaaattttctgggagttcattgactctgccagtcagaatcaatcctgcagtaattctttatttacaggtgaaagtaaaagagaatcccaattttttgcttgtacattaaggtcctccttacattacagctaatttcaaaataagatgaagttggattcgtgtcctttcatggtgatgtgatattctgcactataccaaacaccgtgaaatgtcagctagagcttgtcatgaggcagttgctgccaatcactacatatagatccttcacggagaaaagttggcttcattctctgttgctaatcggctgagcccaggcatcaaataaaacgaaaggctcagtcgaaagactgggcctttcgttttatctgttgtttgtcggtgaacgctctctactagagtcacactggctcaccttcgggtgggcctttctgcgtttatatagagggaaatgtgcgcggaacccctatttgtttatttttctaaatacattcaaatatgtatccgctcatgagacaataaccctgataaatgcttcaataatattgaaaaaggaagagtatgagtattcaacatttccgtgtcgcccttattcccttttttgcggcattttgccttcctgtttttgctcacccagaaacgctggtgaaagtaaaagatgctgaagatcagttgggtgcacgagtgggttacatcgaactggatctcaacagcggtaagatccttgagagttttcgccccgaagaacgttttccaatgatgagcacttttaaagttctgctatgtggcgcggtattatcccgtattgacgccgggcaagagcaactcggtcgccgcatacactattctcagaatgacttggttgagtactcaccagtcacagaaaagcatcttacggatggcatgacagtaagagaattatgcagtgctgccataaccatgagtgataacactgcggccaacttacttctgacaacgatcggaggaccgaaggagctaaccgcttttttgcacaacatgggggatcatgtaactcgccttgatcgttgggaaccggagctgaatgaagccataccaaacgacgagcgtgacaccacgatgcctgtagcaatggcaacaacgttgcgcaaactattaactggcgaactacttactctagcttcccggcaacaattaatagactggatggaggcggataaagttgcaggaccacttctgcgctcggcccttccggctggctggtttattgctgataaatctggagccggtgagcgtgggtcacgcggtatcattgcagcactggggccagatggtaagccctcccgtatcgtagttatctacacgacggggagtcaggcaactatggatgaacgaaatagacagatcgctgagataggtgcctcactgattaagcattggtaactgtcagaccaagtttactcatatatactttagattgatttaaaacttcatttttaatttaaaaggatctaggtgaagatcctttttgataatctcatgaccaaaatcccttaacgtgagttttcgttccactgagcgtcagaccccgtagaaaagatcaaaggatcttcttgagatcctttttttctgcgcgtaatctgctgcttgcaaacaaaaaaaccaccgctaccagcggtggtttgtttgccggatcaagagctaccaactctttttccgaaggtaactggcttcagcagagcgcagataccaaatactgttcttctagtgtagccgtagttaggccaccacttcaagaactctgtagcaccgcctacatacctcgctctgctaatcctgttaccagtggctgctgccagtggcgataagtcgtgtcttaccgggttggactcaagacgatagttaccggataaggcgcagcggtcgggctgaacggggggttcgtgcacacagcccagcttggagcgaacgacctacaccgaactgagatacctacagcgtgagctatgagaaagcgccacgcttcccgaagggagaaaggcggacaggtatccggtaagcggcagggtcggaacaggagagcgcacgagggagcttccagggggaaacgcctggtatctttatagtcctgtcgggtttcgccacctctgacttgagcgtcgatttttgtgatgctcgtcaggggggcggagcctatggaaaaacgccagcaacgcggcctttttacggttcctggccttttgctggccttttgctcacatgttctttcctgcgttatcccctgattctgtggataaccgtattaccgccagagaatataaaaagccagattattaatccggcttttttattatttgacgcgttttgagattcaaaattcaatctgtttggacctggataagacacaagagcgacatcctgacatgaacgccgtaaacagcaaatcctggttgaacacgtatccttttgggggcctcccgctacgacgctcgctccagctggggcttccttactatacacagcgcgcatatttcacggttgccagatgtcaagatggccaagttgaccagtgccgttccggtgctcaccgcgcgcgacgtcgccggagcggtcgagttctggaccgaccggctcgggttctcccgggacttcgtggaggacgacttcgccggtgtggtccgggacgacgtgaccctgttcatcagcgcggtccaggaccaggtggtgccggacaacaccctggcctgggtgtgggtgcgcggcctggacgagctgtacgccgagtggtcggaggtcgtgtccacgaacttccgggacgcctccgggccggccatgaccgagatcggcgagcagccgtgggggcgggagttcgccctgcgcgacccggccggcaactgcgtgcacttcgtggccgaggagcaggactgaaccttccttaaaaatttaattttcattagttgcagtcactccgctttggtttcacagtcaggaataacactagctcgtcttcaccatggatgccaatctcgcctattcatggtgtataaaagttcaacatccaaagctagaacttttggaaagagaaagaatatccgaatagggcacggcgtgccgtattgttggagtggactagcagaaagtgaggaaggcacaggatgagttttctcgatt

SEQ ID NO: 44 - DNA, 6059 bp, artificial
  Vector NVB7
ttcgattggaatggttttggagaggaaaccgtttttatggcggttggatgggaaaggaagggatggtgttcacactcagatttgggagctcacccaccgtatgttgacagtacaaacaatcctgcaatcctgcgaaccaactgtttctcgtctttttggtctgtacgtggtaggatagagagtctgccgggataccatttcgtgcgcagacgtggaagagtcattattcagcttgcacgacacagattttatacagacaaacgtacaatacgcaattgctccgacaaaaattgccgaccattcctacaggcatatttttgcatataattaggggaaacgcatagaatgcaatcttcagttacatacagacaacattctgtcgcagctcgccacacgtaccaactccagattccgagcttcgccgcggccttttggaaagatcgaaaaggcgccgccgcggctgtcgttcccgcagaaagtgcaagcagccactagcgcaaaaatctatggatttccaagtacaaatcttcagttttctacttatctcggccagtgtaataattagtaggggcgacattgtcatgacacaaactcctctatcctcacctgtgacccttggacaacccgcctctatcagctgccgttcctcccaatcgctggtccattccgatggaaacacgtacttgtcttggctccaacagcgccctgggcagcccccgcggctcttgatttataaaataagtaacagatttagcggcgttccggaccggttcagtggttcgggcgcaggtaccgatttcacccttaagatctcccgcgtagaggccgaggatgtaggagtgtattactgtatgcaagcaactcaatttccccaccaatggacgttcggtcaagggactaaagttgaaattaagcgtacggttgctgcgccatccgtctttatttttccgccatctgacgaacagctcaaaagcggaacggcttctgtcgtctgtctcctgaacaatttttacccgcgagaggctaaggttcagtggaaggtcgataatgcgttgcagtcgggcaactcgcaggaatctgtgacggaacaggacagcaaggactccacatacagcttatcgtcgacattgacactgtcaaaagcggactacgagaaacacaaggtgtatgcctgcgaagttacccatcagggattgtcatcaccagtgaccaaatcatttaatcgaggtgaatgcgagggccgagggtcgctcttgacgtgcggtgacgtcgaagaaaacccgggacccatggattttcaggtccaaatattttcttttcttctgatatcagcctctgtcattataagtcggggggaagtccacctcgtggaaagcggggggggtttagtacagccgggtggcgccttgagactctcttgtgcagcctcgggattcaccttttcaaactacgatatgcattgggtgaggcaggccaccggcaagggtctggagtgggtgagtgctaatggcaccgcaggtgatacttattatccaggtagcgtcaaaggccgtttcacgattagtcgcgaaaacgctaagaattctctctatttgcagatgaattcactacgagcaggtgacacagcagtctactattgtgcgagggacgttgatattgttgcgaccatcaccgattacttcgattactggggtcaaggcactttggtaacagtttctagtgcgagtactaagggtccgagtgtatttcctttagccccttcctctaaaagcacttcaggcggaacagcagcccttggctgtttggtgaaagactacttcccggaacctgtaactgtgagctggaattctggcgcgctcactagtggagttcacacttttccagccgtgttacagtcatcgggtctttattccctgtcctccgtcgtgaccgtcccgtcgagttcactaggtacgcagacatacatttgtaacgtcaatcacaagccatcgaacacaaaggtggacaagcgtgttgaacccaagagctgcgataagacccacacctgccctccctgcccagctcccgagcttctcggcggaccttcggttttcctctttccgccgaagcccaaagatactttgatgatttcacggacgccagaagtgacatgcgtggttgttgacgtaagccatgaggatccggaagtgaaatttaactggtacgtcgatggagttgaggtccataacgccaagaccaagccccgcgaggaacaatataattccacatatcgtgtggtgtcggtacttacggtccttcatcaggactggctaaatggaaaagaatacaaatgcaaggtgtccaataaagcgctccccgctcccatcgaaaagacgatcagcaaggcgaaggggcaaccacgtgaaccgcaagtatacacgctcccgccctcccgagaagaaatgacaaaaaaccaagtctccctgacctgtttggttaaaggattttacccttcggacatcgcggtagagtgggagtccaacggacaacctgagaataactacaaaacgactcctccagtcctggactcggacggatccttcttcttgtactccaaattgacggttgacaaatcccgatggcaacaaggcaacgtttttagctgctcggtcatgcatgaagctttgcacaaccactacacacaaaaatcgttgtcgctgtcgccaggaaaataaaaccacggacgtttgttggagattccgcttttacctgatttccagttcctgtaattttgtcgttccttatgtttccacacaaacgactgcaagcaaaatcaactaatttgtttatcacatttcaatagccagtttgaatgtttttcttacgatactgtaggcagtggaagcggaattggtttttgtgggcaaccgaaaaaggcttgcaattttcaattagggtaacagtagtcggtaaacaattgctcatctagctctaggaagtctattaatccacaggttggaaacgcaatgaatgtgccatgtatgacggcgccggtgtaggcaggagaatttctctaatgtaatctttgttccacgactcttacagaggcacccaaaccatcgcttcgatcagttgacgagaggtttctgaaaacgatcttatcgaggcgccgttggtggtcctttcgaaagaatcacttccaacatgtagctttgggatgcaaaactttcattggatgtgagcccaggcatcaaataaaacgaaaggctcagtcgaaagactgggcctttcgttttatctgttgtttgtcggtgaacgctctctactagagtcacactggctcaccttcgggtgggcctttctgcgtttatatagagggaaatgtgcgcggaacccctatttgtttatttttctaaatacattcaaatatgtatccgctcatgagacaataaccctgataaatgcttcaataatattgaaaaaggaagagtatgagtattcaacatttccgtgtcgcccttattcccttttttgcggcattttgccttcctgtttttgctcacccagaaacgctggtgaaagtaaaagatgctgaagatcagttgggtgcacgagtgggttacatcgaactggatctcaacagcggtaagatccttgagagttttcgccccgaagaacgttttccaatgatgagcacttttaaagttctgctatgtggcgcggtattatcccgtattgacgccgggcaagagcaactcggtcgccgcatacactattctcagaatgacttggttgagtactcaccagtcacagaaaagcatcttacggatggcatgacagtaagagaattatgcagtgctgccataaccatgagtgataacactgcggccaacttacttctgacaacgatcggaggaccgaaggagctaaccgcttttttgcacaacatgggggatcatgtaactcgccttgatcgttgggaaccggagctgaatgaagccataccaaacgacgagcgtgacaccacgatgcctgtagcaatggcaacaacgttgcgcaaactattaactggcgaactacttactctagcttcccggcaacaattaatagactggatggaggcggataaagttgcaggaccacttctgcgctcggcccttccggctggctggtttattgctgataaatctggagccggtgagcgtgggtcacgcggtatcattgcagcactggggccagatggtaagccctcccgtatcgtagttatctacacgacggggagtcaggcaactatggatgaacgaaatagacagatcgctgagataggtgcctcactgattaagcattggtaactgtcagaccaagtttactcatatatactttagattgatttaaaacttcatttttaatttaaaaggatctaggtgaagatcctttttgataatctcatgaccaaaatcccttaacgtgagttttcgttccactgagcgtcagaccccgtagaaaagatcaaaggatcttcttgagatcctttttttctgcgcgtaatctgctgcttgcaaacaaaaaaaccaccgctaccagcggtggtttgtttgccggatcaagagctaccaactctttttccgaaggtaactggcttcagcagagcgcagataccaaatactgttcttctagtgtagccgtagttaggccaccacttcaagaactctgtagcaccgcctacatacctcgctctgctaatcctgttaccagtggctgctgccagtggcgataagtcgtgtcttaccgggttggactcaagacgatagttaccggataaggcgcagcggtcgggctgaacggggggttcgtgcacacagcccagcttggagcgaacgacctacaccgaactgagatacctacagcgtgagctatgagaaagcgccacgcttcccgaagggagaaaggcggacaggtatccggtaagcggcagggtcggaacaggagagcgcacgagggagcttccagggggaaacgcctggtatctttatagtcctgtcgggtttcgccacctctgacttgagcgtcgatttttgtgatgctcgtcaggggggcggagcctatggaaaaacgccagcaacgcggcctttttacggttcctggccttttgctggccttttgctcacatgttctttcctgcgttatcccctgattctgtggataaccgtattaccgccagagaatataaaaagccagattattaatccggcttttttattatttgacgcgttttgagattcaaaattcaatctgtttggacctggataagacacaagagcgacatcctgacatgaacgccgtaaacagcaaatcctggttgaacacgtatccttttgggggcctcccgctacgacgctcgctccagctggggcttccttactatacacagcgcgcatatttcacggttgccagatgtcaagatggccaagttgaccagtgccgttccggtgctcaccgcgcgcgacgtcgccggagcggtcgagttctggaccgaccggctcgggttctcccgggacttcgtggaggacgacttcgccggtgtggtccgggacgacgtgaccctgttcatcagcgcggtccaggaccaggtggtgccggacaacaccctggcctgggtgtgggtgcgcggcctggacgagctgtacgccgagtggtcggaggtcgtgtccacgaacttccgggacgcctccgggccggccatgaccgagatcggcgagcagccgtgggggcgggagttcgccctgcgcgacccggccggcaactgcgtgcacttcgtggccgaggagcaggactgaaccttccttaaaaatttaattttcattagttgcagtcactccgctttggtttcacagtcaggaataacactagctcgtcttcaccatggatgccaatctcgcctattcatggtgtataaaagttcaacatccaaagctagaacttttggaaagagaaagaatatccgaatagggcacggcgtgccgtattgttggagtggactagcagaaagtgaggaaggcacaggatgagttttctcgatt

SEQ ID NO: 45 - DNA, 5748 bp, artificial
  Vector C
catatgcggaagtgactgtaaacgagaagtgcacgaagccttttcttgtgacgtcacaaaccgaacagccctacgtggcgtgcgactttccggcactttggatatcgttgccctatatgtattgggtgtatacatgtcgtattccaactacgacagaaaacagtcagttacgggtattcgaacttccggcacctgcagcgaggagttttgtgtccgtcgcacatcctccgtgctttcggcacctacgtaggcggcaaacttcctgccttccgcccgccttgcggcattccggctccgggccagaattgcccgggtgttcacaattttgcctcctcacgaaaaaacgttctactttgtattttggtcgggtttcggatccttccagcaaccattctcattcaaagtcaccacttgtgcgaacgtatcatggattttcaggtccaaatattttcttttcttctgatatcagcctctgtcattataagtcggggggaagtccacctcgtggaaagcggggggggtttagtacagccgggtggcgccttgagactctcttgtgcagcctcgggattcaccttttcaaactacgatatgcattgggtgaggcaggccaccggcaagggtctggagtgggtgagtgctaatggcaccgcaggtgatacttattatccaggtagcgtcaaaggccgtttcacgattagtcgcgaaaacgctaagaattctctctatttgcagatgaattcactacgagcaggtgacacagcagtctactattgtgcgagggacgttgatattgttgcgaccatcaccgattacttcgattactggggtcaaggcactttggtaacagtttctagtgcgagtactaagggtccgagtgtatttcctttagccccttcctctaaaagcacttcaggcggaacagcagcccttggctgtttggtgaaagactacttcccggaacctgtaactgtgagctggaattctggcgcgctcactagtggagttcacacttttccagccgtgttacagtcatcgggtctttattccctgtcctccgtcgtgaccgtcccgtcgagttcactaggtacgcagacatacatttgtaacgtcaatcacaagccatcgaacacaaaggtggacaagcgtgttgaacccaagagctgcgataagacccacacctgccctccctgcccagctcccgagcttctcggcggaccttcggttttcctctttccgccgaagcccaaagatactttgatgatttcacggacgccagaagtgacatgcgtggttgttgacgtaagccatgaggatccggaagtgaaatttaactggtacgtcgatggagttgaggtccataacgccaagaccaagccccgcgaggaacaatataattccacatatcgtgtggtgtcggtacttacggtccttcatcaggactggctaaatggaaaagaatacaaatgcaaggtgtccaataaagcgctccccgctcccatcgaaaagacgatcagcaaggcgaaggggcaaccacgtgaaccgcaagtatacacgctcccgccctcccgagaagaaatgacaaaaaaccaagtctccctgacctgtttggttaaaggattttacccttcggacatcgcggtagagtgggagtccaacggacaacctgagaataactacaaaacgactcctccagtcctggactcggacggatccttcttcttgtactccaaattgacggttgacaaatcccgatggcaacaaggcaacgtttttagctgctcggtcatgcatgaagctttgcacaaccactacacacaaaaatcgttgtcgctgtcgccaggaaaagagggccgagggtcgctcttgacgtgcggtgacgtcgaagaaaacccgggacccatggatttccaagtacaaatcttcagttttctacttatctcggccagtgtaataattagtaggggcgacattgtcatgacacaaactcctctatcctcacctgtgacccttggacaacccgcctctatcagctgccgttcctcccaatcgctggtccattccgatggaaacacgtacttgtcttggctccaacagcgccctgggcagcccccgcggctcttgatttataaaataagtaacagatttagcggcgttccggaccggttcagtggttcgggcgcaggtaccgatttcacccttaagatctcccgcgtagaggccgaggatgtaggagtgtattactgtatgcaagcaactcaatttccccaccaatggacgttcggtcaagggactaaagttgaaattaagcgtacggttgctgcgccatccgtctttatttttccgccatctgacgaacagctcaaaagcggaacggcttctgtcgtctgtctcctgaacaatttttacccgcgagaggctaaggttcagtggaaggtcgataatgcgttgcagtcgggcaactcgcaggaatctgtgacggaacaggacagcaaggactccacatacagcttatcgtcgacattgacactgtcaaaagcggactacgagaaacacaaggtgtatgcctgcgaagttacccatcagggattgtcatcaccagtgaccaaatcatttaatcgaggtgaatgctaagtaacaatttactttaagactagcgcaatttttttcttacattagatgaacataaaacgacgatgaggatcactgttagggaaacgatgaactacgctgaggacttcctattattcgtcctttgatggcgtggttgttctttggtttgcggccgagcgcaacgaccaaggcctgtaccaaaaacgaagttgataatcagatatttgagttgtaacaagaaactaaagcattattttagcagtagcacggatcaggatctaaaatgaacgcatccggaccaggcatcaaataaaacgaaaggctcagtcgaaagactgggcctttcgttttatctgttgtttgtcggtgaacgctctctactagagtcacactggctcaccttcgggtgggcctttctgcgtttatatagagggaaatgtgcgcggaacccctatttgtttatttttctaaatacattcaaatatgtatccgctcatgagacaataaccctgataaatgcttcaataatattgaaaaaggaagagtatgagtattcaacatttccgtgtcgcccttattcccttttttgcggcattttgccttcctgtttttgctcacccagaaacgctggtgaaagtaaaagatgctgaagatcagttgggtgcacgagtgggttacatcgaactggatctcaacagcggtaagatccttgagagttttcgccccgaagaacgttttccaatgatgagcacttttaaagttctgctatgtggcgcggtattatcccgtattgacgccgggcaagagcaactcggtcgccgcatacactattctcagaatgacttggttgagtactcaccagtcacagaaaagcatcttacggatggcatgacagtaagagaattatgcagtgctgccataaccatgagtgataacactgcggccaacttacttctgacaacgatcggaggaccgaaggagctaaccgcttttttgcacaacatgggggatcatgtaactcgccttgatcgttgggaaccggagctgaatgaagccataccaaacgacgagcgtgacaccacgatgcctgtagcaatggcaacaacgttgcgcaaactattaactggcgaactacttactctagcttcccggcaacaattaatagactggatggaggcggataaagttgcaggaccacttctgcgctcggcccttccggctggctggtttattgctgataaatctggagccggtgagcgtgggtcacgcggtatcattgcagcactggggccagatggtaagccctcccgtatcgtagttatctacacgacggggagtcaggcaactatggatgaacgaaatagacagatcgctgagataggtgcctcactgattaagcattggtaactgtcagaccaagtttactcatatatactttagattgatttaaaacttcatttttaatttaaaaggatctaggtgaagatcctttttgataatctcatgaccaaaatcccttaacgtgagttttcgttccactgagcgtcagaccccgtagaaaagatcaaaggatcttcttgagatcctttttttctgcgcgtaatctgctgcttgcaaacaaaaaaaccgctaccagcggtggtttgtttgccggatcaagagctaccaactctttttccgaaggtaactggcttcagcagagcgcagataccaaatactgttcttctagtgtagccgtagttaggccaccacttcaagaactctgtagcaccgcctacatacctcgctctgctaatcctgttaccagtggctgctgccagtggcgataagtcgtgtcttaccgggttggactcaagacgatagttaccggataaggcgcagcggtcgggctgaacggggggttcgtgcacacagcccagcttggagcgaacgacctacaccgaactgagatacctacagcgtgagctatgagaaagcgccacgcttcccgaagggagaaaggcggacaggtatccggtaagcggcagggtcggaacaggagagcgcacgagggagcttccagggggaaacgcctggtatctttatagtcctgtcgggtttcgccacctctgacttgagcgtcgatttttgtgatgctcgtcaggggggcggagcctatggaaaaacgccagcaacgcggcctttttacggttcctggccttttgctggccttttgctcacatgttctttcctgcgttatcccctgattctgtggataaccgtattaccgccagagaatataaaaagccagattattaatccggcttttttattatttgacgcgttttgagattcaaaattcaatctgtttggacctggataagacacaagagcgacatcctgacatgaacgccgtaaacagcaaatcctggttgaacacgtatccttttgggggcctccgctacgacgctcgctccagctggggcttccttactatacacagcgcgcatatttcacggttgccagatgtcaagatggccaagttgaccagtgccgttccggtgctcaccgcgcgcgacgtcgccggagcggtcgagttctggaccgaccggctcgggttctcccgggacttcgtggaggacgacttcgccggtgtggtccgggacgacgtgaccctgttcatcagcgcggtccaggaccaggtggtgccggacaacaccctggcctgggtgtgggtgcgcggcctggacgagctgtacgccgagtggtcggaggtcgtgtccacgaacttccgggacgcctccgggccggccatgaccgagatcggcgagcagccgtgggggcgggagttcgccctgcgcgacccggccggcaactgcgtgcacttcgtggccgaggagcaggactgaaccttccttaaaaatttaattttcattagttgcagtcactccgctttggtttcacagtcaggaataacactagctcgtcttcaccatggatgccaatctcgcctattcatggtgtataaaagttcaacatccaaagctagaacttttggaaagagaaagaatatccgaatagggcacggcgtgccgtattgttggagtggactagcagaaagtgaggaaggcacaggatgagttttctcgaaagacg

SEQ ID NO: 46 - DNA, 5748 bp, artificial
  Vector D
catatgcggaagtgactgtaaacgagaagtgcacgaagccttttcttgtgacgtcacaaaccgaacagccctacgtggcgtgcgactttccggcactttggatatcgttgccctatatgtattgggtgtatacatgtcgtattccaactacgacagaaaacagtcagttacgggtattcgaacttccggcacctgcagcgaggagttttgtgtccgtcgcacatcctccgtgctttcggcacctacgtaggcggcaaacttcctgccttccgcccgccttgcggcattccggctccgggccagaattgcccgggtgttcacaattttgcctcctcacgaaaaaacgttctactttgtattttggtcgggtttcggatccttccagcaaccattctcattcaaagtcaccacttgtgcgaacgtatcatggatttccaagtacaaatcttcagttttctacttatctcggccagtgtaataattagtaggggcgacattgtcatgacacaaactcctctatcctcacctgtgacccttggacaacccgcctctatcagctgccgttcctcccaatcgctggtccattccgatggaaacacgtacttgtcttggctccaacagcgccctgggcagcccccgcggctcttgatttataaaataagtaacagatttagcggcgttccggaccggttcagtggttcgggcgcaggtaccgatttcacccttaagatctcccgcgtagaggccgaggatgtaggagtgtattactgtatgcaagcaactcaatttccccaccaatggacgttcggtcaagggactaaagttgaaattaagcgtacggttgctgcgccatccgtctttatttttccgccatctgacgaacagctcaaaagcggaacggcttctgtcgtctgtctcctgaacaatttttacccgcgagaggctaaggttcagtggaaggtcgataatgcgttgcagtcgggcaactcgcaggaatctgtgacggaacaggacagcaaggactccacatacagcttatcgtcgacattgacactgtcaaaagcggactacgagaaacacaaggtgtatgcctgcgaagttacccatcagggattgtcatcaccagtgaccaaatcatttaatcgaggtgaatgcgagggccgagggtcgctcttgacgtgcggtgacgtcgaagaaaacccgggacccatggattttcaggtccaaatattttcttttcttctgatatcagcctctgtcattataagtcggggggaagtccacctcgtggaaagcggggggggtttagtacagccgggtggcgccttgagactctcttgtgcagcctcgggattcaccttttcaaactacgatatgcattgggtgaggcaggccaccggcaagggtctggagtgggtgagtgctaatggcaccgcaggtgatacttattatccaggtagcgtcaaaggccgtttcacgattagtcgcgaaaacgctaagaattctctctatttgcagatgaattcactacgagcaggtgacacagcagtctactattgtgcgagggacgttgatattgttgcgaccatcaccgattacttcgattactggggtcaaggcactttggtaacagtttctagtgcgagtactaagggtccgagtgtatttcctttagccccttcctctaaaagcacttcaggcggaacagcagcccttggctgtttggtgaaagactacttcccggaacctgtaactgtgagctggaattctggcgcgctcactagtggagttcacacttttccagccgtgttacagtcatcgggtctttattccctgtcctccgtcgtgaccgtcccgtcgagttcactaggtacgcagacatacatttgtaacgtcaatcacaagccatcgaacacaaaggtggacaagcgtgttgaacccaagagctgcgataagacccacacctgccctccctgcccagctcccgagcttctcggcggaccttcggttttcctctttccgccgaagcccaaagatactttgatgatttcacggacgccagaagtgacatgcgtggttgttgacgtaagccatgaggatccggaagtgaaatttaactggtacgtcgatggagttgaggtccataacgccaagaccaagccccgcgaggaacaatataattccacatatcgtgtggtgtcggtacttacggtccttcatcaggactggctaaatggaaaagaatacaaatgcaaggtgtccaataaagcgctccccgctcccatcgaaaagacgatcagcaaggcgaaggggcaaccacgtgaaccgcaagtatacacgctcccgccctcccgagaagaaatgacaaaaaaccaagtctccctgacctgtttggttaaaggattttacccttcggacatcgcggtagagtgggagtccaacggacaacctgagaataactacaaaacgactcctccagtcctggactcggacggatccttcttcttgtactccaaattgacggttgacaaatcccgatggcaacaaggcaacgtttttagctgctcggtcatgcatgaagctttgcacaaccactacacacaaaaatcgttgtcgctgtcgccaggaaaataagtaacaatttactttaagactagcgcaatttttttcttacattagatgaacataaaacgacgatgaggatcactgttagggaaacgatgaactacgctgaggacttcctattattcgtcctttgatggcgtggttgttctttggtttgcggccgagcgcaacgaccaaggcctgtaccaaaaacgaagttgataatcagatatttgagttgtaacaagaaactaaagcattattttagcagtagcacggatcaggatctaaaatgaacgcatccggaccaggcatcaaataaaacgaaaggctcagtcgaaagactgggcctttcgttttatctgttgtttgtcggtgaacgctctctactagagtcacactggctcaccttcgggtgggcctttctgcgtttatatagagggaaatgtgcgcggaacccctatttgtttatttttctaaatacattcaaatatgtatccgctcatgagacaataaccctgataaatgcttcaataatattgaaaaaggaagagtatgagtattcaacatttccgtgtcgcccttattcccttttttgcggcattttgccttcctgtttttgctcacccagaaacgctggtgaaagtaaaagatgctgaagatcagttgggtgcacgagtgggttacatcgaactggatctcaacagcggtaagatccttgagagttttcgccccgaagaacgttttccaatgatgagcacttttaaagttctgctatgtggcgcggtattatcccgtattgacgccgggcaagagcaactcggtcgccgcatacactattctcagaatgacttggttgagtactcaccagtcacagaaaagcatcttacggatggcatgacagtaagagaattatgcagtgctgccataaccatgagtgataacactgcggccaacttacttctgacaacgatcggaggaccgaaggagctaaccgcttttttgcacaacatgggggatcatgtaactcgccttgatcgttgggaaccggagctgaatgaagccataccaaacgacgagcgtgacaccacgatgcctgtagcaatggcaacaacgttgcgcaaactattaactggcgaactacttactctagcttcccggcaacaattaatagactggatggaggcggataaagttgcaggaccacttctgcgctcggcccttccggctggctggtttattgctgataaatctggagccggtgagcgtgggtcacgcggtatcattgcagcactggggccagatggtaagccctcccgtatcgtagttatctacacgacggggagtcaggcaactatggatgaacgaaatagacagatcgctgagataggtgcctcactgattaagcattggtaactgtcagaccaagtttactcatatatactttagattgatttaaaacttcatttttaatttaaaaggatctaggtgaagatcctttttgataatctcatgaccaaaatcccttaacgtgagttttcgttccactgagcgtcagaccccgtagaaaagatcaaaggatcttcttgagatcctttttttctgcgcgtaatctgctgcttgcaaacaaaaaaaccgctaccagcggtggtttgtttgccggatcaagagctaccaactctttttccgaaggtaactggcttcagcagagcgcagataccaaatactgttcttctagtgtagccgtagttaggccaccacttcaagaactctgtagcaccgcctacatacctcgctctgctaatcctgttaccagtggctgctgccagtggcgataagtcgtgtcttaccgggttggactcaagacgatagttaccggataaggcgcagcggtcgggctgaacggggggttcgtgcacacagcccagcttggagcgaacgacctacaccgaactgagatacctacagcgtgagctatgagaaagcgccacgcttcccgaagggagaaaggcggacaggtatccggtaagcggcagggtcggaacaggagagcgcacgagggagcttccagggggaaacgcctggtatctttatagtcctgtcgggtttcgccacctctgacttgagcgtcgatttttgtgatgctcgtcaggggggcggagcctatggaaaaacgccagcaacgcggcctttttacggttcctggccttttgctggccttttgctcacatgttctttcctgcgttatcccctgattctgtggataaccgtattaccgccagagaatataaaaagccagattattaatccggcttttttattatttgacgcgttttgagattcaaaattcaatctgtttggacctggataagacacaagagcgacatcctgacatgaacgccgtaaacagcaaatcctggttgaacacgtatccttttgggggcctccgctacgacgctcgctccagctggggcttccttactatacacagcgcgcatatttcacggttgccagatgtcaagatggccaagttgaccagtgccgttccggtgctcaccgcgcgcgacgtcgccggagcggtcgagttctggaccgaccggctcgggttctcccgggacttcgtggaggacgacttcgccggtgtggtccgggacgacgtgaccctgttcatcagcgcggtccaggaccaggtggtgccggacaacaccctggcctgggtgtgggtgcgcggcctggacgagctgtacgccgagtggtcggaggtcgtgtccacgaacttccgggacgcctccgggccggccatgaccgagatcggcgagcagccgtgggggcgggagttcgccctgcgcgacccggccggcaactgcgtgcacttcgtggccgaggagcaggactgaaccttccttaaaaatttaattttcattagttgcagtcactccgctttggtttcacagtcaggaataacactagctcgtcttcaccatggatgccaatctcgcctattcatggtgtataaaagttcaacatccaaagctagaacttttggaaagagaaagaatatccgaatagggcacggcgtgccgtattgttggagtggactagcagaaagtgaggaaggcacaggatgagttttctcgaaagacg

SEQ ID NO: 47 - DNA, 6570 bp, artificial
  Vector Pro1D
tttttgtcgctacttcaccacagctttattgaatagggacgagcttttattaatcatgtgctgctgtcctttttgcatcaggattgtcacgtagccactttggactgtaattaatcttgacttctttatctaacaaagcggcgagatcaaggtccttctcagtcaaaccctgcagcttgtgtgtccaaatttttacctcgatatctcggtaactagtaagatggaagtcggggtggtgactttcgcgttcagctatggcccccatctcgttgatgcattttaaagcagactgaaaattgcgtgccgtaaatttacgagatatatgcaaaggttctgattcactcgagcaaagattccacagcgatccccttatcccaagtttgtccactgcactttcaaatgtcaatagaaaagatgcgtccagagtagagcaaggagcgcaatgtttcggtccttgcggggagcctgaagccatcactaatactgtgaaaatgagagccggcaatttctgaagactatgtaagtctccgaacaggaaggaagcgcaagcaaaccacaattcgaactccagataaacttgctgttagcacaatcaacatgaccatgtacaagcgtcgtctgcttgtgagcccgtcaatatgattgattgagggcagatccttagcactttaaccctgtaaacatttttgttttggctctcatcaacggcagctgtagcgaatctatagcctgccgggcagtataacgttcatgatcaaaaatgaagtgtatataagtcgataaatgtaaccctttttcttgctatataattttttttgaacgatgaacactaaacacacatagctatctgacatcgaacataaatgtaagagtcattccaaataagtagagatgcaatgtggacatcatgggatgatgtgtggatttacgatcccctcaactgtaaaactattcttaggcacaatttaccgagcgaacaaaaatactaaagaaacttagcatattttcgaaagcattgtaattttcaacctttgtgaaattttttctatattttccgaagtgtgacagtgaattccaaatcttgagtctgctttgtgtactttgacatgacaactttcggacacgctcactttttgacgaccacacgttcaatcgttgctgcgctccggcacagactaaagttcaggaattgcttgtcacctacgcagcatcaccactctctcgtctctaccgtgattcaaggctgaatcatggatttccaagtacaaatcttcagttttctacttatctcggccagtgtaataattagtaggggcgacattgtcatgacacaaactcctctatcctcacctgtgacccttggacaacccgcctctatcagctgccgttcctcccaatcgctggtccattccgatggaaacacgtacttgtcttggctccaacagcgccctgggcagcccccgcggctcttgatttataaaataagtaacagatttagcggcgttccggaccggttcagtggttcgggcgcaggtaccgatttcacccttaagatctcccgcgtagaggccgaggatgtaggagtgtattactgtatgcaagcaactcaatttccccaccaatggacgttcggtcaagggactaaagttgaaattaagcgtacggttgctgcgccatccgtctttatttttccgccatctgacgaacagctcaaaagcggaacggcttctgtcgtctgtctcctgaacaatttttacccgcgagaggctaaggttcagtggaaggtcgataatgcgttgcagtcgggcaactcgcaggaatctgtgacggaacaggacagcaaggactccacatacagcttatcgtcgacattgacactgtcaaaagcggactacgagaaacacaaggtgtatgcctgcgaagttacccatcagggattgtcatcaccagtgaccaaatcatttaatcgaggtgaatgcgagggccgagggtcgctcttgacgtgcggtgacgtcgaagaaaacccgggacccatggattttcaggtccaaatattttcttttcttctgatatcagcctctgtcattataagtcggggggaagtccacctcgtggaaagcggggggggtttagtacagccgggtggcgccttgagactctcttgtgcagcctcgggattcaccttttcaaactacgatatgcattgggtgaggcaggccaccggcaagggtctggagtgggtgagtgctaatggcaccgcaggtgatacttattatccaggtagcgtcaaaggccgtttcacgattagtcgcgaaaacgctaagaattctctctatttgcagatgaattcactacgagcaggtgacacagcagtctactattgtgcgagggacgttgatattgttgcgaccatcaccgattacttcgattactggggtcaaggcactttggtaacagtttctagtgcgagtactaagggtccgagtgtatttcctttagccccttcctctaaaagcacttcaggcggaacagcagcccttggctgtttggtgaaagactacttcccggaacctgtaactgtgagctggaattctggcgcgctcactagtggagttcacacttttccagccgtgttacagtcatcgggtctttattccctgtcctccgtcgtgaccgtcccgtcgagttcactaggtacgcagacatacatttgtaacgtcaatcacaagccatcgaacacaaaggtggacaagcgtgttgaacccaagagctgcgataagacccacacctgccctccctgcccagctcccgagcttctcggcggaccttcggttttcctctttccgccgaagcccaaagatactttgatgatttcacggacgccagaagtgacatgcgtggttgttgacgtaagccatgaggatccggaagtgaaatttaactggtacgtcgatggagttgaggtccataacgccaagaccaagccccgcgaggaacaatataattccacatatcgtgtggtgtcggtacttacggtccttcatcaggactggctaaatggaaaagaatacaaatgcaaggtgtccaataaagcgctccccgctcccatcgaaaagacgatcagcaaggcgaaggggcaaccacgtgaaccgcaagtatacacgctcccgccctcccgagaagaaatgacaaaaaaccaagtctccctgacctgtttggttaaaggattttacccttcggacatcgcggtagagtgggagtccaacggacaacctgagaataactacaaaacgactcctccagtcctggactcggacggatccttcttcttgtactccaaattgacggttgacaaatcccgatggcaacaaggcaacgtttttagctgctcggtcatgcatgaagctttgcacaaccactacacacaaaaatcgttgtcgctgtcgccaggaaaataaaacccaatttactttaagactagcgcaatttttttcttacattagatgaacataaaacgacgatgaggatcactgttagggaaacgatgaactacgctgaggacttcctattattcgtcctttgatggcgtggttgttctttggtttgcggccgagcgcaacgaccaaggcctgtaccaaaaacgaagttgataatcagatatttgagttgtaacaagaaactaaagcattattttagcagtagcacgaatcaggatctaaaatgaacgcatccggaccaggcatcaaataaaacgaaaggctcagtcgaaagactgggcctttcgttttatctgttgtttgtcggtgaacgctctctactagagtcacactggctcaccttcgggtgggcctttctgcgtttatatagagggaaatgtgcgcggaacccctatttgtttatttttctaaatacattcaaatatgtatccgctcatgagacaataaccctgataaatgcttcaataatattgaaaaaggaagagtatgagtattcaacatttccgtgtcgcccttattcccttttttgcggcattttgccttcctgtttttgctcacccagaaacgctggtgaaagtaaaagatgctgaagatcagttgggtgcacgagtgggttacatcgaactggatctcaacagcggtaagatccttgagagttttcgccccgaagaacgttttccaatgatgagcacttttaaagttctgctatgtggcgcggtattatcccgtattgacgccgggcaagagcaactcggtcgccgcatacactattctcagaatgacttggttgagtactcaccagtcacagaaaagcatcttacggatggcatgacagtaagagaattatgcagtgctgccataaccatgagtgataacactgcggccaacttacttctgacaacgatcggaggaccgaaggagctaaccgcttttttgcacaacatgggggatcatgtaactcgccttgatcgttgggaaccggagctgaatgaagccataccaaacgacgagcgtgacaccacgatgcctgtagcaatggcaacaacgttgcgcaaactattaactggcgaactacttactctagcttcccggcaacaattaatagactggatggaggcggataaagttgcaggaccacttctgcgctcggcccttccggctggctggtttattgctgataaatctggagccggtgagcgtgggtcacgcggtatcattgcagcactggggccagatggtaagccctcccgtatcgtagttatctacacgacggggagtcaggcaactatggatgaacgaaatagacagatcgctgagataggtgcctcactgattaagcattggtaactgtcagaccaagtttactcatatatactttagattgatttaaaacttcatttttaatttaaaaggatctaggtgaagatcctttttgataatctcatgaccaaaatcccttaacgtgagttttcgttccactgagcgtcagaccccgtagaaaagatcaaaggatcttcttgagatcctttttttctgcgcgtaatctgctgcttgcaaacaaaaaaaccaccgctaccagcggtggtttgtttgccggatcaagagctaccaactctttttccgaaggtaactggcttcagcagagcgcagataccaaatactgttcttctagtgtagccgtagttaggccaccacttcaagaactctgtagcaccgcctacatacctcgctctgctaatcctgttaccagtggctgctgccagtggcgataagtcgtgtcttaccgggttggactcaagacgatagttaccggataaggcgcagcggtcgggctgaacggggggttcgtgcacacagcccagcttggagcgaacgacctacaccgaactgagatacctacagcgtgagctatgagaaagcgccacgcttcccgaagggagaaaggcggacaggtatccggtaagcggcagggtcggaacaggagagcgcacgagggagcttccagggggaaacgcctggtatctttatagtcctgtcgggtttcgccacctctgacttgagcgtcgatttttgtgatgctcgtcaggggggcggagcctatggaaaaacgccagcaacgcggcctttttacggttcctggccttttgctggccttttgctcacatgttctttcctgcgttatcccctgattctgtggataaccgtattaccgccagagaatataaaaagccagattattaatccggcttttttattatttgacgcgttttgagattcaaaattcaatctgtttggacctggataagacacaagagcgacatcctgacatgaacgccgtaaacagcaaatcctggttgaacacgtatccttttgggggcctcccgctacgacgctcgctccagctggggcttccttactatacacagcgcgcatatttcacggttgccagatgtcaagatggccaagttgaccagtgccgttccggtgctcaccgcgcgcgacgtcgccggagcggtcgagttctggaccgaccggctcgggttctcccgggacttcgtggaggacgacttcgccggtgtggtccgggacgacgtgaccctgttcatcagcgcggtccaggaccaggtggtgccggacaacaccctggcctgggtgtgggtgcgcggcctggacgagctgtacgccgagtggtcggaggtcgtgtccacgaacttccgggacgcctccgggccggccatgaccgagatcggcgagcagccgtgggggcgggagttcgccctgcgcgacccggccggcaactgcgtgcacttcgtggccgaggagcaggactgaaccttccttaaaaatttaattttcattagttgcagtcactccgctttggtttcacagtcaggaataacactagctcgtcttcaccatggatgccaatctcgcctattcatggtgtataaaagttcaacatccaaagctagaacttttggaaagagaaagaatatccgaatagggcacggcgtgccgtattgttggagtggactagcagaaagtgaggaaggcacaggatgagttttctcga

SEQ ID NO: 48 - DNA, 6449 bp, artificial
  Vector Pro2D
tttttcgggttggagtactgctaggagcaccataagccaaagactatgtgctgctggtgaactctaaaagcggacggcaattaacggtttgtgtttcttaaccattgtcatgatggtggtcgtcgaggttgtttctcgtcgttgttagcaagattcaaccctgcatctcggtataaagtgcgcaatgcgtctacagcaactcaccatcaatctgcgatcttgttcgttcgcaagaccacgaaatttgctggccttcaggaaaggaaaatactgttggtctatatccgagtcttggagtagggcaacacgacaatgctgtgctgtatatgaagtcagacaacacaccacaaacccatactcccaaataaatgtatagcgatttatcgaaagagctcggttcaaagaatttgtccaaacatggtcggaaatattccaaaagcgacaaaggctaagtaagctaagtcctcttggtgcttgaaaggaaagctgcagaggggatgatttaaaattacgcgaaaggaaggagcttctaagatggagagagagagagaccgcagtcatgtttacaaagtgaagctacaaaatggccagaacaaatgatgtactattttggctacgtgtaggtggaccggtcctattggccaaatgagcccaaacagaaccctagccacaatttttttactaattaagctgtggtctttcttatgcgtcaggtgggtttcatttctcgaagaacgttttcgctccccgaggcggtcttgctccattagtcaatgatgtcacgcataccatattcctgcgactaccgtctcaaataaagccggtaacgcaacaatatgtaggctgatgttatggtgtgatttaacaaggcccaaacagttttttaacaggttactattggcgattcaagacatcacaataatgaccatcttaaacgattcagagtgtgactcatccgggaaagtagggtcgcatgtttcctgagagaatcgcttcatgagatctcatcggttgcaactggtctcacaagtgaacgttagataagcaataacagcaaacctttgtgatttcagctaactgtgaccagatcgcttctagactggaaacaactctcatccattccacgactatggatttccaagtacaaatcttcagttttctacttatctcggccagtgtaataattagtaggggcgacattgtcatgacacaaactcctctatcctcacctgtgacccttggacaacccgcctctatcagctgccgttcctcccaatcgctggtccattccgatggaaacacgtacttgtcttggctccaacagcgccctgggcagcccccgcggctcttgatttataaaataagtaacagatttagcggcgttccggaccggttcagtggttcgggcgcaggtaccgatttcacccttaagatctcccgcgtagaggccgaggatgtaggagtgtattactgtatgcaagcaactcaatttccccaccaatggacgttcggtcaagggactaaagttgaaattaagcgtacggttgctgcgccatccgtctttatttttccgccatctgacgaacagctcaaaagcggaacggcttctgtcgtctgtctcctgaacaatttttacccgcgagaggctaaggttcagtggaaggtcgataatgcgttgcagtcgggcaactcgcaggaatctgtgacggaacaggacagcaaggactccacatacagcttatcgtcgacattgacactgtcaaaagcggactacgagaaacacaaggtgtatgcctgcgaagttacccatcagggattgtcatcaccagtgaccaaatcatttaatcgaggtgaatgcgagggccgagggtcgctcttgacgtgcggtgacgtcgaagaaaacccgggacccatggattttcaggtccaaatattttcttttcttctgatatcagcctctgtcattataagtcggggggaagtccacctcgtggaaagcggggggggtttagtacagccgggtggcgccttgagactctcttgtgcagcctcgggattcaccttttcaaactacgatatgcattgggtgaggcaggccaccggcaagggtctggagtgggtgagtgctaatggcaccgcaggtgatacttattatccaggtagcgtcaaaggccgtttcacgattagtcgcgaaaacgctaagaattctctctatttgcagatgaattcactacgagcaggtgacacagcagtctactattgtgcgagggacgttgatattgttgcgaccatcaccgattacttcgattactggggtcaaggcactttggtaacagtttctagtgcgagtactaagggtccgagtgtatttcctttagccccttcctctaaaagcacttcaggcggaacagcagcccttggctgtttggtgaaagactacttcccggaacctgtaactgtgagctggaattctggcgcgctcactagtggagttcacacttttccagccgtgttacagtcatcgggtctttattccctgtcctccgtcgtgaccgtcccgtcgagttcactaggtacgcagacatacatttgtaacgtcaatcacaagccatcgaacacaaaggtggacaagcgtgttgaacccaagagctgcgataagacccacacctgccctccctgcccagctcccgagcttctcggcggaccttcggttttcctctttccgccgaagcccaaagatactttgatgatttcacggacgccagaagtgacatgcgtggttgttgacgtaagccatgaggatccggaagtgaaatttaactggtacgtcgatggagttgaggtccataacgccaagaccaagccccgcgaggaacaatataattccacatatcgtgtggtgtcggtacttacggtccttcatcaggactggctaaatggaaaagaatacaaatgcaaggtgtccaataaagcgctccccgctcccatcgaaaagacgatcagcaaggcgaaggggcaaccacgtgaaccgcaagtatacacgctcccgccctcccgagaagaaatgacaaaaaaccaagtctccctgacctgtttggttaaaggattttacccttcggacatcgcggtagagtgggagtccaacggacaacctgagaataactacaaaacgactcctccagtcctggactcggacggatccttcttcttgtactccaaattgacggttgacaaatcccgatggcaacaaggcaacgtttttagctgctcggtcatgcatgaagctttgcacaaccactacacacaaaaatcgttgtcgctgtcgccaggaaaataaaacccaatttactttaagactagcgcaatttttttcttacattagatgaacataaaacgacgatgaggatcactgttagggaaacgatgaactacgctgaggacttcctattattcgtcctttgatggcgtggttgttctttggtttgcggccgagcgcaacgaccaaggcctgtaccaaaaacgaagttgataatcagatatttgagttgtaacaagaaactaaagcattattttagcagtagcacgaatcaggatctaaaatgaacgcatccggaccaggcatcaaataaaacgaaaggctcagtcgaaagactgggcctttcgttttatctgttgtttgtcggtgaacgctctctactagagtcacactggctcaccttcgggtgggcctttctgcgtttatatagagggaaatgtgcgcggaacccctatttgtttatttttctaaatacattcaaatatgtatccgctcatgagacaataaccctgataaatgcttcaataatattgaaaaaggaagagtatgagtattcaacatttccgtgtcgcccttattcccttttttgcggcattttgccttcctgtttttgctcacccagaaacgctggtgaaagtaaaagatgctgaagatcagttgggtgcacgagtgggttacatcgaactggatctcaacagcggtaagatccttgagagttttcgccccgaagaacgttttccaatgatgagcacttttaaagttctgctatgtggcgcggtattatcccgtattgacgccgggcaagagcaactcggtcgccgcatacactattctcagaatgacttggttgagtactcaccagtcacagaaaagcatcttacggatggcatgacagtaagagaattatgcagtgctgccataaccatgagtgataacactgcggccaacttacttctgacaacgatcggaggaccgaaggagctaaccgcttttttgcacaacatgggggatcatgtaactcgccttgatcgttgggaaccggagctgaatgaagccataccaaacgacgagcgtgacaccacgatgcctgtagcaatggcaacaacgttgcgcaaactattaactggcgaactacttactctagcttcccggcaacaattaatagactggatggaggcggataaagttgcaggaccacttctgcgctcggcccttccggctggctggtttattgctgataaatctggagccggtgagcgtgggtcacgcggtatcattgcagcactggggccagatggtaagccctcccgtatcgtagttatctacacgacggggagtcaggcaactatggatgaacgaaatagacagatcgctgagataggtgcctcactgattaagcattggtaactgtcagaccaagtttactcatatatactttagattgatttaaaacttcatttttaatttaaaaggatctaggtgaagatcctttttgataatctcatgaccaaaatcccttaacgtgagttttcgttccactgagcgtcagaccccgtagaaaagatcaaaggatcttcttgagatcctttttttctgcgcgtaatctgctgcttgcaaacaaaaaaaccaccgctaccagcggtggtttgtttgccggatcaagagctaccaactctttttccgaaggtaactggcttcagcagagcgcagataccaaatactgttcttctagtgtagccgtagttaggccaccacttcaagaactctgtagcaccgcctacatacctcgctctgctaatcctgttaccagtggctgctgccagtggcgataagtcgtgtcttaccgggttggactcaagacgatagttaccggataaggcgcagcggtcgggctgaacggggggttcgtgcacacagcccagcttggagcgaacgacctacaccgaactgagatacctacagcgtgagctatgagaaagcgccacgcttcccgaagggagaaaggcggacaggtatccggtaagcggcagggtcggaacaggagagcgcacgagggagcttccagggggaaacgcctggtatctttatagtcctgtcgggtttcgccacctctgacttgagcgtcgatttttgtgatgctcgtcaggggggcggagcctatggaaaaacgccagcaacgcggcctttttacggttcctggccttttgctggccttttgctcacatgttctttcctgcgttatcccctgattctgtggataaccgtattaccgccagagaatataaaaagccagattattaatccggcttttttattatttgacgcgttttgagattcaaaattcaatctgtttggacctggataagacacaagagcgacatcctgacatgaacgccgtaaacagcaaatcctggttgaacacgtatccttttgggggcctcccgctacgacgctcgctccagctggggcttccttactatacacagcgcgcatatttcacggttgccagatgtcaagatggccaagttgaccagtgccgttccggtgctcaccgcgcgcgacgtcgccggagcggtcgagttctggaccgaccggctcgggttctcccgggacttcgtggaggacgacttcgccggtgtggtccgggacgacgtgaccctgttcatcagcgcggtccaggaccaggtggtgccggacaacaccctggcctgggtgtgggtgcgcggcctggacgagctgtacgccgagtggtcggaggtcgtgtccacgaacttccgggacgcctccgggccggccatgaccgagatcggcgagcagccgtgggggcgggagttcgccctgcgcgacccggccggcaactgcgtgcacttcgtggccgaggagcaggactgaaccttccttaaaaatttaattttcattagttgcagtcactccgctttggtttcacagtcaggaataacactagctcgtcttcaccatggatgccaatctcgcctattcatggtgtataaaagttcaacatccaaagctagaacttttggaaagagaaagaatatccgaatagggcacggcgtgccgtattgttggagtggactagcagaaagtgaggaaggcacaggatgagttttctcga

SEQ ID NO: 49 - DNA, 5859 bp, artificial
  Vector Pro3D
tttttaattatcattgtatgttcgttctctaggaatttatagtcaagcttccttttgctactaccctgctcctcaatcagcgtcagggaagcaagatcctcctcggctagggtcttagcatggttcttggcctacgctagctaggaaggtaccataaaaacgagagctattaatggctcagcatttatccgatacatgtttaacagaaagacagaaaacacgaaaaaagttgttgacagtgaatgctccagatgtcacaagaaaggcgttggggcgaatcgattgggcctttggaggcattagtaaaaaggagaaagctttttaatctttgtcgacatgtacttctatacaatattgctatagaattgaaggacagcttgaaatgtctatcgacatagtgactccgacttaaggtcattcactatttttacgcgtgaccgcggacccaaaacccgaccggcagttcctgccccaaacataatacaaattatagctccaaaattgactctctttgaaccgacgacccaattggttctaccatggatttccaagtacaaatcttcagttttctacttatctcggccagtgtaataattagtaggggcgacattgtcatgacacaaactcctctatcctcacctgtgacccttggacaacccgcctctatcagctgccgttcctcccaatcgctggtccattccgatggaaacacgtacttgtcttggctccaacagcgccctgggcagcccccgcggctcttgatttataaaataagtaacagatttagcggcgttccggaccggttcagtggttcgggcgcaggtaccgatttcacccttaagatctcccgcgtagaggccgaggatgtaggagtgtattactgtatgcaagcaactcaatttccccaccaatggacgttcggtcaagggactaaagttgaaattaagcgtacggttgctgcgccatccgtctttatttttccgccatctgacgaacagctcaaaagcggaacggcttctgtcgtctgtctcctgaacaatttttacccgcgagaggctaaggttcagtggaaggtcgataatgcgttgcagtcgggcaactcgcaggaatctgtgacggaacaggacagcaaggactccacatacagcttatcgtcgacattgacactgtcaaaagcggactacgagaaacacaaggtgtatgcctgcgaagttacccatcagggattgtcatcaccagtgaccaaatcatttaatcgaggtgaatgcgagggccgagggtcgctcttgacgtgcggtgacgtcgaagaaaacccgggacccatggattttcaggtccaaatattttcttttcttctgatatcagcctctgtcattataagtcggggggaagtccacctcgtggaaagcggggggggtttagtacagccgggtggcgccttgagactctcttgtgcagcctcgggattcaccttttcaaactacgatatgcattgggtgaggcaggccaccggcaagggtctggagtgggtgagtgctaatggcaccgcaggtgatacttattatccaggtagcgtcaaaggccgtttcacgattagtcgcgaaaacgctaagaattctctctatttgcagatgaattcactacgagcaggtgacacagcagtctactattgtgcgagggacgttgatattgttgcgaccatcaccgattacttcgattactggggtcaaggcactttggtaacagtttctagtgcgagtactaagggtccgagtgtatttcctttagccccttcctctaaaagcacttcaggcggaacagcagcccttggctgtttggtgaaagactacttcccggaacctgtaactgtgagctggaattctggcgcgctcactagtggagttcacacttttccagccgtgttacagtcatcgggtctttattccctgtcctccgtcgtgaccgtcccgtcgagttcactaggtacgcagacatacatttgtaacgtcaatcacaagccatcgaacacaaaggtggacaagcgtgttgaacccaagagctgcgataagacccacacctgccctccctgcccagctcccgagcttctcggcggaccttcggttttcctctttccgccgaagcccaaagatactttgatgatttcacggacgccagaagtgacatgcgtggttgttgacgtaagccatgaggatccggaagtgaaatttaactggtacgtcgatggagttgaggtccataacgccaagaccaagccccgcgaggaacaatataattccacatatcgtgtggtgtcggtacttacggtccttcatcaggactggctaaatggaaaagaatacaaatgcaaggtgtccaataaagcgctccccgctcccatcgaaaagacgatcagcaaggcgaaggggcaaccacgtgaaccgcaagtatacacgctcccgccctcccgagaagaaatgacaaaaaaccaagtctccctgacctgtttggttaaaggattttacccttcggacatcgcggtagagtgggagtccaacggacaacctgagaataactacaaaacgactcctccagtcctggactcggacggatccttcttcttgtactccaaattgacggttgacaaatcccgatggcaacaaggcaacgtttttagctgctcggtcatgcatgaagctttgcacaaccactacacacaaaaatcgttgtcgctgtcgccaggaaaataaaacccaatttactttaagactagcgcaatttttttcttacattagatgaacataaaacgacgatgaggatcactgttagggaaacgatgaactacgctgaggacttcctattattcgtcctttgatggcgtggttgttctttggtttgcggccgagcgcaacgaccaaggcctgtaccaaaaacgaagttgataatcagatatttgagttgtaacaagaaactaaagcattattttagcagtagcacgaatcaggatctaaaatgaacgcatccggaccaggcatcaaataaaacgaaaggctcagtcgaaagactgggcctttcgttttatctgttgtttgtcggtgaacgctctctactagagtcacactggctcaccttcgggtgggcctttctgcgtttatatagagggaaatgtgcgcggaacccctatttgtttatttttctaaatacattcaaatatgtatccgctcatgagacaataaccctgataaatgcttcaataatattgaaaaaggaagagtatgagtattcaacatttccgtgtcgcccttattcccttttttgcggcattttgccttcctgtttttgctcacccagaaacgctggtgaaagtaaaagatgctgaagatcagttgggtgcacgagtgggttacatcgaactggatctcaacagcggtaagatccttgagagttttcgccccgaagaacgttttccaatgatgagcacttttaaagttctgctatgtggcgcggtattatcccgtattgacgccgggcaagagcaactcggtcgccgcatacactattctcagaatgacttggttgagtactcaccagtcacagaaaagcatcttacggatggcatgacagtaagagaattatgcagtgctgccataaccatgagtgataacactgcggccaacttacttctgacaacgatcggaggaccgaaggagctaaccgcttttttgcacaacatgggggatcatgtaactcgccttgatcgttgggaaccggagctgaatgaagccataccaaacgacgagcgtgacaccacgatgcctgtagcaatggcaacaacgttgcgcaaactattaactggcgaactacttactctagcttcccggcaacaattaatagactggatggaggcggataaagttgcaggaccacttctgcgctcggcccttccggctggctggtttattgctgataaatctggagccggtgagcgtgggtcacgcggtatcattgcagcactggggccagatggtaagccctcccgtatcgtagttatctacacgacggggagtcaggcaactatggatgaacgaaatagacagatcgctgagataggtgcctcactgattaagcattggtaactgtcagaccaagtttactcatatatactttagattgatttaaaacttcatttttaatttaaaaggatctaggtgaagatcctttttgataatctcatgaccaaaatcccttaacgtgagttttcgttccactgagcgtcagaccccgtagaaaagatcaaaggatcttcttgagatcctttttttctgcgcgtaatctgctgcttgcaaacaaaaaaaccaccgctaccagcggtggtttgtttgccggatcaagagctaccaactctttttccgaaggtaactggcttcagcagagcgcagataccaaatactgttcttctagtgtagccgtagttaggccaccacttcaagaactctgtagcaccgcctacatacctcgctctgctaatcctgttaccagtggctgctgccagtggcgataagtcgtgtcttaccgggttggactcaagacgatagttaccggataaggcgcagcggtcgggctgaacggggggttcgtgcacacagcccagcttggagcgaacgacctacaccgaactgagatacctacagcgtgagctatgagaaagcgccacgcttcccgaagggagaaaggcggacaggtatccggtaagcggcagggtcggaacaggagagcgcacgagggagcttccagggggaaacgcctggtatctttatagtcctgtcgggtttcgccacctctgacttgagcgtcgatttttgtgatgctcgtcaggggggcggagcctatggaaaaacgccagcaacgcggcctttttacggttcctggccttttgctggccttttgctcacatgttctttcctgcgttatcccctgattctgtggataaccgtattaccgccagagaatataaaaagccagattattaatccggcttttttattatttgacgcgttttgagattcaaaattcaatctgtttggacctggataagacacaagagcgacatcctgacatgaacgccgtaaacagcaaatcctggttgaacacgtatccttttgggggcctcccgctacgacgctcgctccagctggggcttccttactatacacagcgcgcatatttcacggttgccagatgtcaagatggccaagttgaccagtgccgttccggtgctcaccgcgcgcgacgtcgccggagcggtcgagttctggaccgaccggctcgggttctcccgggacttcgtggaggacgacttcgccggtgtggtccgggacgacgtgaccctgttcatcagcgcggtccaggaccaggtggtgccggacaacaccctggcctgggtgtgggtgcgcggcctggacgagctgtacgccgagtggtcggaggtcgtgtccacgaacttccgggacgcctccgggccggccatgaccgagatcggcgagcagccgtgggggcgggagttcgccctgcgcgacccggccggcaactgcgtgcacttcgtggccgaggagcaggactgaaccttccttaaaaatttaattttcattagttgcagtcactccgctttggtttcacagtcaggaataacactagctcgtcttcaccatggatgccaatctcgcctattcatggtgtataaaagttcaacatccaaagctagaacttttggaaagagaaagaatatccgaatagggcacggcgtgccgtattgttggagtggactagcagaaagtgaggaaggcacaggatgagttttctcga

SEQ ID NO: 50 - DNA, 6419 bp, artificial
  Vector pro4D
ttttaaattgtatactccagcagtcgtttaataccggagacggtagacgcaagagcagctcacactctttggccacgactgtaaatgcctctagtgttgacgagtttgcgtgcacgagagaaattttcgagagaacacaggaaggaccccagtacttttgggtccttttgagcttgcaacgcttttcgtttcgaaaaccaaatccaaatccctttcgacacaggggctttttctcgcgcatgtgataaaaagcaaacaaaacccggagatcatccaaggtcgtcactgtcagaatacggtgactctagaaggcaatgcggaactcccagccggccgcatactattgacgatgaatcatcttgcttttcattactataggttgttggccgcctctcgatttattttcgagtgatctgtttaaaatgttcctcattcggtgaattttcttgcagaccatgtcccaagtcctacactaccacagcagatgatggaattaaggtcaccgtcaaaaggtagacagagtcgcgttagaaaccatgttagataaagggtcaaacggaatgttgcggattccccagggctatagacaggactaccaaagagatctgcgatcaaaattttgttgcacagcacatataccgaaagataacttgagttatccttacattgggagtcccaaaaatcaatctttcgagcgtcttcgtgccgcaacaattagatggccagttggaacaaaaaaagtatcaaatggtcgaaaatacccaagagaaacgctcactaatagaattctgtctgcctcttatatttctttgaacatgagcgttattagcaggtaaacagttgtttcgtaaatctgacattaatagtggagtgtggtcataatgccgcgctcctctgatgtcgaaactatggattcattgaaaacggtcatcggtcatagcaaaggaacttcgctttctagtaaataaccacacaaacaaatttcctcacctctttcgttgaatctggcatttccatcaacaccttttcatagctttgtggatggattgagttgcgctcgctgtcaccatttgcgccgaattccttgccctttacagtaatggatttccaagtacaaatcttcagttttctacttatctcggccagtgtaataattagtaggggcgacattgtcatgacacaaactcctctatcctcacctgtgacccttggacaacccgcctctatcagctgccgttcctcccaatcgctggtccattccgatggaaacacgtacttgtcttggctccaacagcgccctgggcagcccccgcggctcttgatttataaaataagtaacagatttagcggcgttccggaccggttcagtggttcgggcgcaggtaccgatttcacccttaagatctcccgcgtagaggccgaggatgtaggagtgtattactgtatgcaagcaactcaatttccccaccaatggacgttcggtcaagggactaaagttgaaattaagcgtacggttgctgcgccatccgtctttatttttccgccatctgacgaacagctcaaaagcggaacggcttctgtcgtctgtctcctgaacaatttttacccgcgagaggctaaggttcagtggaaggtcgataatgcgttgcagtcgggcaactcgcaggaatctgtgacggaacaggacagcaaggactccacatacagcttatcgtcgacattgacactgtcaaaagcggactacgagaaacacaaggtgtatgcctgcgaagttacccatcagggattgtcatcaccagtgaccaaatcatttaatcgaggtgaatgcgagggccgagggtcgctcttgacgtgcggtgacgtcgaagaaaacccgggacccatggattttcaggtccaaatattttcttttcttctgatatcagcctctgtcattataagtcggggggaagtccacctcgtggaaagcggggggggtttagtacagccgggtggcgccttgagactctcttgtgcagcctcgggattcaccttttcaaactacgatatgcattgggtgaggcaggccaccggcaagggtctggagtgggtgagtgctaatggcaccgcaggtgatacttattatccaggtagcgtcaaaggccgtttcacgattagtcgcgaaaacgctaagaattctctctatttgcagatgaattcactacgagcaggtgacacagcagtctactattgtgcgagggacgttgatattgttgcgaccatcaccgattacttcgattactggggtcaaggcactttggtaacagtttctagtgcgagtactaagggtccgagtgtatttcctttagccccttcctctaaaagcacttcaggcggaacagcagcccttggctgtttggtgaaagactacttcccggaacctgtaactgtgagctggaattctggcgcgctcactagtggagttcacacttttccagccgtgttacagtcatcgggtctttattccctgtcctccgtcgtgaccgtcccgtcgagttcactaggtacgcagacatacatttgtaacgtcaatcacaagccatcgaacacaaaggtggacaagcgtgttgaacccaagagctgcgataagacccacacctgccctccctgcccagctcccgagcttctcggcggaccttcggttttcctctttccgccgaagcccaaagatactttgatgatttcacggacgccagaagtgacatgcgtggttgttgacgtaagccatgaggatccggaagtgaaatttaactggtacgtcgatggagttgaggtccataacgccaagaccaagccccgcgaggaacaatataattccacatatcgtgtggtgtcggtacttacggtccttcatcaggactggctaaatggaaaagaatacaaatgcaaggtgtccaataaagcgctccccgctcccatcgaaaagacgatcagcaaggcgaaggggcaaccacgtgaaccgcaagtatacacgctcccgccctcccgagaagaaatgacaaaaaaccaagtctccctgacctgtttggttaaaggattttacccttcggacatcgcggtagagtgggagtccaacggacaacctgagaataactacaaaacgactcctccagtcctggactcggacggatccttcttcttgtactccaaattgacggttgacaaatcccgatggcaacaaggcaacgtttttagctgctcggtcatgcatgaagctttgcacaaccactacacacaaaaatcgttgtcgctgtcgccaggaaaataaaacccaatttactttaagactagcgcaatttttttcttacattagatgaacataaaacgacgatgaggatcactgttagggaaacgatgaactacgctgaggacttcctattattcgtcctttgatggcgtggttgttctttggtttgcggccgagcgcaacgaccaaggcctgtaccaaaaacgaagttgataatcagatatttgagttgtaacaagaaactaaagcattattttagcagtagcacgaatcaggatctaaaatgaacgcatccggaccaggcatcaaataaaacgaaaggctcagtcgaaagactgggcctttcgttttatctgttgtttgtcggtgaacgctctctactagagtcacactggctcaccttcgggtgggcctttctgcgtttatatagagggaaatgtgcgcggaacccctatttgtttatttttctaaatacattcaaatatgtatccgctcatgagacaataaccctgataaatgcttcaataatattgaaaaaggaagagtatgagtattcaacatttccgtgtcgcccttattcccttttttgcggcattttgccttcctgtttttgctcacccagaaacgctggtgaaagtaaaagatgctgaagatcagttgggtgcacgagtgggttacatcgaactggatctcaacagcggtaagatccttgagagttttcgccccgaagaacgttttccaatgatgagcacttttaaagttctgctatgtggcgcggtattatcccgtattgacgccgggcaagagcaactcggtcgccgcatacactattctcagaatgacttggttgagtactcaccagtcacagaaaagcatcttacggatggcatgacagtaagagaattatgcagtgctgccataaccatgagtgataacactgcggccaacttacttctgacaacgatcggaggaccgaaggagctaaccgcttttttgcacaacatgggggatcatgtaactcgccttgatcgttgggaaccggagctgaatgaagccataccaaacgacgagcgtgacaccacgatgcctgtagcaatggcaacaacgttgcgcaaactattaactggcgaactacttactctagcttcccggcaacaattaatagactggatggaggcggataaagttgcaggaccacttctgcgctcggcccttccggctggctggtttattgctgataaatctggagccggtgagcgtgggtcacgcggtatcattgcagcactggggccagatggtaagccctcccgtatcgtagttatctacacgacggggagtcaggcaactatggatgaacgaaatagacagatcgctgagataggtgcctcactgattaagcattggtaactgtcagaccaagtttactcatatatactttagattgatttaaaacttcatttttaatttaaaaggatctaggtgaagatcctttttgataatctcatgaccaaaatcccttaacgtgagttttcgttccactgagcgtcagaccccgtagaaaagatcaaaggatcttcttgagatcctttttttctgcgcgtaatctgctgcttgcaaacaaaaaaaccaccgctaccagcggtggtttgtttgccggatcaagagctaccaactctttttccgaaggtaactggcttcagcagagcgcagataccaaatactgttcttctagtgtagccgtagttaggccaccacttcaagaactctgtagcaccgcctacatacctcgctctgctaatcctgttaccagtggctgctgccagtggcgataagtcgtgtcttaccgggttggactcaagacgatagttaccggataaggcgcagcggtcgggctgaacggggggttcgtgcacacagcccagcttggagcgaacgacctacaccgaactgagatacctacagcgtgagctatgagaaagcgccacgcttcccgaagggagaaaggcggacaggtatccggtaagcggcagggtcggaacaggagagcgcacgagggagcttccagggggaaacgcctggtatctttatagtcctgtcgggtttcgccacctctgacttgagcgtcgatttttgtgatgctcgtcaggggggcggagcctatggaaaaacgccagcaacgcggcctttttacggttcctggccttttgctggccttttgctcacatgttctttcctgcgttatcccctgattctgtggataaccgtattaccgccagagaatataaaaagccagattattaatccggcttttttattatttgacgcgttttgagattcaaaattcaatctgtttggacctggataagacacaagagcgacatcctgacatgaacgccgtaaacagcaaatcctggttgaacacgtatccttttgggggcctcccgctacgacgctcgctccagctggggcttccttactatacacagcgcgcatatttcacggttgccagatgtcaagatggccaagttgaccagtgccgttccggtgctcaccgcgcgcgacgtcgccggagcggtcgagttctggaccgaccggctcgggttctcccgggacttcgtggaggacgacttcgccggtgtggtccgggacgacgtgaccctgttcatcagcgcggtccaggaccaggtggtgccggacaacaccctggcctgggtgtgggtgcgcggcctggacgagctgtacgccgagtggtcggaggtcgtgtccacgaacttccgggacgcctccgggccggccatgaccgagatcggcgagcagccgtgggggcgggagttcgccctgcgcgacccggccggcaactgcgtgcacttcgtggccgaggagcaggactgaaccttccttaaaaatttaattttcattagttgcagtcactccgctttggtttcacagtcaggaataacactagctcgtcttcaccatggatgccaatctcgcctattcatggtgtataaaagttcaacatccaaagctagaacttttggaaagagaaagaatatccgaatagggcacggcgtgccgtattgttggagtggactagcagaaagtgaggaaggcacaggatgagttttctcga

SEQ ID NO: 51 - DNA, 6281 bp, artificial
  Vector pro5D
ttttaatcataggcaatgtttggtacacaataaatttgacgtagttcattatgtgctgcaatactgaatacttgccaggagtgacaggattctagctcctgaggagcgcttacagtggaattacacacatgacttgtaccgacagccaactaactataataagaagcaatgcggacttggtaggatcctttcatcaattcaaacattcactatcaatcaaaaattacaaattttacttgcttgcagtcagcatatatttgtcaacgcattgggttctttcatagtcaaatagaaatgtcacgagaatagctcccgggcccgtcaagttcttaattctgtaacttgtccttgccactccatttgcacttgacgtatcacttgtcgctctcaacacagcattacacaatggcactctacagagcattggttaatgtaaattattgaaaggcaaaacatagcccttcttgactgtgagtcccaccatcgctacgagtcacttacatgtaaaatatctgtccttccatcgagggcacggaattctgaaacgaaaacaatcttgttgggctcggtagtccgttacgcaaaaacgcttctatcaattcaattaggattggtcttggtttggagctgcccgacgcgctcaaaaattgactgggtatgggtacactttctctctgtcgaaatattttgtacagtcattttggttcttgggtatgcttattggagatgatcagttgatgcgcgacggattgagcccaaacaatttacatcatagagatatgcactttggaaaagaccctctgcggtcatctgcaaatcccacaagctttttgctctcgaaccttcacaatcttacccgagttgctatcgttgctagcagcctttcccattgattgccaacattttgatcctgacaacccatagattcgctctgttaaaccaacagcaacagcaagcaaatatggatttccaagtacaaatcttcagttttctacttatctcggccagtgtaataattagtaggggcgacattgtcatgacacaaactcctctatcctcacctgtgacccttggacaacccgcctctatcagctgccgttcctcccaatcgctggtccattccgatggaaacacgtacttgtcttggctccaacagcgccctgggcagcccccgcggctcttgatttataaaataagtaacagatttagcggcgttccggaccggttcagtggttcgggcgcaggtaccgatttcacccttaagatctcccgcgtagaggccgaggatgtaggagtgtattactgtatgcaagcaactcaatttccccaccaatggacgttcggtcaagggactaaagttgaaattaagcgtacggttgctgcgccatccgtctttatttttccgccatctgacgaacagctcaaaagcggaacggcttctgtcgtctgtctcctgaacaatttttacccgcgagaggctaaggttcagtggaaggtcgataatgcgttgcagtcgggcaactcgcaggaatctgtgacggaacaggacagcaaggactccacatacagcttatcgtcgacattgacactgtcaaaagcggactacgagaaacacaaggtgtatgcctgcgaagttacccatcagggattgtcatcaccagtgaccaaatcatttaatcgaggtgaatgcgagggccgagggtcgctcttgacgtgcggtgacgtcgaagaaaacccgggacccatggattttcaggtccaaatattttcttttcttctgatatcagcctctgtcattataagtcggggggaagtccacctcgtggaaagcggggggggtttagtacagccgggtggcgccttgagactctcttgtgcagcctcgggattcaccttttcaaactacgatatgcattgggtgaggcaggccaccggcaagggtctggagtgggtgagtgctaatggcaccgcaggtgatacttattatccaggtagcgtcaaaggccgtttcacgattagtcgcgaaaacgctaagaattctctctatttgcagatgaattcactacgagcaggtgacacagcagtctactattgtgcgagggacgttgatattgttgcgaccatcaccgattacttcgattactggggtcaaggcactttggtaacagtttctagtgcgagtactaagggtccgagtgtatttcctttagccccttcctctaaaagcacttcaggcggaacagcagcccttggctgtttggtgaaagactacttcccggaacctgtaactgtgagctggaattctggcgcgctcactagtggagttcacacttttccagccgtgttacagtcatcgggtctttattccctgtcctccgtcgtgaccgtcccgtcgagttcactaggtacgcagacatacatttgtaacgtcaatcacaagccatcgaacacaaaggtggacaagcgtgttgaacccaagagctgcgataagacccacacctgccctccctgcccagctcccgagcttctcggcggaccttcggttttcctctttccgccgaagcccaaagatactttgatgatttcacggacgccagaagtgacatgcgtggttgttgacgtaagccatgaggatccggaagtgaaatttaactggtacgtcgatggagttgaggtccataacgccaagaccaagccccgcgaggaacaatataattccacatatcgtgtggtgtcggtacttacggtccttcatcaggactggctaaatggaaaagaatacaaatgcaaggtgtccaataaagcgctccccgctcccatcgaaaagacgatcagcaaggcgaaggggcaaccacgtgaaccgcaagtatacacgctcccgccctcccgagaagaaatgacaaaaaaccaagtctccctgacctgtttggttaaaggattttacccttcggacatcgcggtagagtgggagtccaacggacaacctgagaataactacaaaacgactcctccagtcctggactcggacggatccttcttcttgtactccaaattgacggttgacaaatcccgatggcaacaaggcaacgtttttagctgctcggtcatgcatgaagctttgcacaaccactacacacaaaaatcgttgtcgctgtcgccaggaaaataaaacccaatttactttaagactagcgcaatttttttcttacattagatgaacataaaacgacgatgaggatcactgttagggaaacgatgaactacgctgaggacttcctattattcgtcctttgatggcgtggttgttctttggtttgcggccgagcgcaacgaccaaggcctgtaccaaaaacgaagttgataatcagatatttgagttgtaacaagaaactaaagcattattttagcagtagcacgaatcaggatctaaaatgaacgcatccggaccaggcatcaaataaaacgaaaggctcagtcgaaagactgggcctttcgttttatctgttgtttgtcggtgaacgctctctactagagtcacactggctcaccttcgggtgggcctttctgcgtttatatagagggaaatgtgcgcggaacccctatttgtttatttttctaaatacattcaaatatgtatccgctcatgagacaataaccctgataaatgcttcaataatattgaaaaaggaagagtatgagtattcaacatttccgtgtcgcccttattcccttttttgcggcattttgccttcctgtttttgctcacccagaaacgctggtgaaagtaaaagatgctgaagatcagttgggtgcacgagtgggttacatcgaactggatctcaacagcggtaagatccttgagagttttcgccccgaagaacgttttccaatgatgagcacttttaaagttctgctatgtggcgcggtattatcccgtattgacgccgggcaagagcaactcggtcgccgcatacactattctcagaatgacttggttgagtactcaccagtcacagaaaagcatcttacggatggcatgacagtaagagaattatgcagtgctgccataaccatgagtgataacactgcggccaacttacttctgacaacgatcggaggaccgaaggagctaaccgcttttttgcacaacatgggggatcatgtaactcgccttgatcgttgggaaccggagctgaatgaagccataccaaacgacgagcgtgacaccacgatgcctgtagcaatggcaacaacgttgcgcaaactattaactggcgaactacttactctagcttcccggcaacaattaatagactggatggaggcggataaagttgcaggaccacttctgcgctcggcccttccggctggctggtttattgctgataaatctggagccggtgagcgtgggtcacgcggtatcattgcagcactggggccagatggtaagccctcccgtatcgtagttatctacacgacggggagtcaggcaactatggatgaacgaaatagacagatcgctgagataggtgcctcactgattaagcattggtaactgtcagaccaagtttactcatatatactttagattgatttaaaacttcatttttaatttaaaaggatctaggtgaagatcctttttgataatctcatgaccaaaatcccttaacgtgagttttcgttccactgagcgtcagaccccgtagaaaagatcaaaggatcttcttgagatcctttttttctgcgcgtaatctgctgcttgcaaacaaaaaaaccaccgctaccagcggtggtttgtttgccggatcaagagctaccaactctttttccgaaggtaactggcttcagcagagcgcagataccaaatactgttcttctagtgtagccgtagttaggccaccacttcaagaactctgtagcaccgcctacatacctcgctctgctaatcctgttaccagtggctgctgccagtggcgataagtcgtgtcttaccgggttggactcaagacgatagttaccggataaggcgcagcggtcgggctgaacggggggttcgtgcacacagcccagcttggagcgaacgacctacaccgaactgagatacctacagcgtgagctatgagaaagcgccacgcttcccgaagggagaaaggcggacaggtatccggtaagcggcagggtcggaacaggagagcgcacgagggagcttccagggggaaacgcctggtatctttatagtcctgtcgggtttcgccacctctgacttgagcgtcgatttttgtgatgctcgtcaggggggcggagcctatggaaaaacgccagcaacgcggcctttttacggttcctggccttttgctggccttttgctcacatgttctttcctgcgttatcccctgattctgtggataaccgtattaccgccagagaatataaaaagccagattattaatccggcttttttattatttgacgcgttttgagattcaaaattcaatctgtttggacctggataagacacaagagcgacatcctgacatgaacgccgtaaacagcaaatcctggttgaacacgtatccttttgggggcctcccgctacgacgctcgctccagctggggcttccttactatacacagcgcgcatatttcacggttgccagatgtcaagatggccaagttgaccagtgccgttccggtgctcaccgcgcgcgacgtcgccggagcggtcgagttctggaccgaccggctcgggttctcccgggacttcgtggaggacgacttcgccggtgtggtccgggacgacgtgaccctgttcatcagcgcggtccaggaccaggtggtgccggacaacaccctggcctgggtgtgggtgcgcggcctggacgagctgtacgccgagtggtcggaggtcgtgtccacgaacttccgggacgcctccgggccggccatgaccgagatcggcgagcagccgtgggggcgggagttcgccctgcgcgacccggccggcaactgcgtgcacttcgtggccgaggagcaggactgaaccttccttaaaaatttaattttcattagttgcagtcactccgctttggtttcacagtcaggaataacactagctcgtcttcaccatggatgccaatctcgcctattcatggtgtataaaagttcaacatccaaagctagaacttttggaaagagaaagaatatccgaatagggcacggcgtgccgtattgttggagtggactagcagaaagtgaggaaggcacaggatgagttttctcga

SEQ ID NO: 52 - DNA, 6196 bp, artificial
  Vector Pro6D
ttttgttgaaactacattgttgtcggatgactcgccgactgcgatacgatagattggtgatcgggcgatcggcaatgaaagacagcccgctgcgattgcagcttggcgtgctctccgtgtggtagactagtgaagcaacgaggaagcggccaaagagcttgtgaaaggtgggcatcgaatcaaaggaatagctaattgtatttccacttcaagaagaaaagatacaactgagcgattgtcactatacttttcaagttggagagcagttgtcactggattttgtctccctactagaaccgacggtcgaagatctgactggtgcgatgtgcacgagaaaaatatcataccggttggtagtcttttgaaatgtctctttggatttgaaagcgaatcgagatttttatcacagtcaattttagtttgtttcggttagatagaactgtaaacttgaacaattgtaaataatcattgagacataagttccgtcggaaatactttaagcagtttgtgtgcaaacatgtacaaacatttacttacttatatctactgtcgcatggagattttgcgttcttgtcttttagttttgcttcccgcttatgcttcttagttcaagttgtgaaacagtgccatacttcttcagcaggatactaacataaatcgattttctttcccccttacagttaataggtcaaatggaagtagtcatcattttcatggcatcgcgctggctaccgagacatttcaggaatcggttgaagtaataaaacttgaaaacccgaataaactgctctggcatcttggcgagtttcgcaagcacttacatctcacaacagcaatactcgtttcctccgttgtgtagaaacaagcctagagaatatggatttccaagtacaaatcttcagttttctacttatctcggccagtgtaataattagtaggggcgacattgtcatgacacaaactcctctatcctcacctgtgacccttggacaacccgcctctatcagctgccgttcctcccaatcgctggtccattccgatggaaacacgtacttgtcttggctccaacagcgccctgggcagcccccgcggctcttgatttataaaataagtaacagatttagcggcgttccggaccggttcagtggttcgggcgcaggtaccgatttcacccttaagatctcccgcgtagaggccgaggatgtaggagtgtattactgtatgcaagcaactcaatttccccaccaatggacgttcggtcaagggactaaagttgaaattaagcgtacggttgctgcgccatccgtctttatttttccgccatctgacgaacagctcaaaagcggaacggcttctgtcgtctgtctcctgaacaatttttacccgcgagaggctaaggttcagtggaaggtcgataatgcgttgcagtcgggcaactcgcaggaatctgtgacggaacaggacagcaaggactccacatacagcttatcgtcgacattgacactgtcaaaagcggactacgagaaacacaaggtgtatgcctgcgaagttacccatcagggattgtcatcaccagtgaccaaatcatttaatcgaggtgaatgcgagggccgagggtcgctcttgacgtgcggtgacgtcgaagaaaacccgggacccatggattttcaggtccaaatattttcttttcttctgatatcagcctctgtcattataagtcggggggaagtccacctcgtggaaagcggggggggtttagtacagccgggtggcgccttgagactctcttgtgcagcctcgggattcaccttttcaaactacgatatgcattgggtgaggcaggccaccggcaagggtctggagtgggtgagtgctaatggcaccgcaggtgatacttattatccaggtagcgtcaaaggccgtttcacgattagtcgcgaaaacgctaagaattctctctatttgcagatgaattcactacgagcaggtgacacagcagtctactattgtgcgagggacgttgatattgttgcgaccatcaccgattacttcgattactggggtcaaggcactttggtaacagtttctagtgcgagtactaagggtccgagtgtatttcctttagccccttcctctaaaagcacttcaggcggaacagcagcccttggctgtttggtgaaagactacttcccggaacctgtaactgtgagctggaattctggcgcgctcactagtggagttcacacttttccagccgtgttacagtcatcgggtctttattccctgtcctccgtcgtgaccgtcccgtcgagttcactaggtacgcagacatacatttgtaacgtcaatcacaagccatcgaacacaaaggtggacaagcgtgttgaacccaagagctgcgataagacccacacctgccctccctgcccagctcccgagcttctcggcggaccttcggttttcctctttccgccgaagcccaaagatactttgatgatttcacggacgccagaagtgacatgcgtggttgttgacgtaagccatgaggatccggaagtgaaatttaactggtacgtcgatggagttgaggtccataacgccaagaccaagccccgcgaggaacaatataattccacatatcgtgtggtgtcggtacttacggtccttcatcaggactggctaaatggaaaagaatacaaatgcaaggtgtccaataaagcgctccccgctcccatcgaaaagacgatcagcaaggcgaaggggcaaccacgtgaaccgcaagtatacacgctcccgccctcccgagaagaaatgacaaaaaaccaagtctccctgacctgtttggttaaaggattttacccttcggacatcgcggtagagtgggagtccaacggacaacctgagaataactacaaaacgactcctccagtcctggactcggacggatccttcttcttgtactccaaattgacggttgacaaatcccgatggcaacaaggcaacgtttttagctgctcggtcatgcatgaagctttgcacaaccactacacacaaaaatcgttgtcgctgtcgccaggaaaataaaacccaatttactttaagactagcgcaatttttttcttacattagatgaacataaaacgacgatgaggatcactgttagggaaacgatgaactacgctgaggacttcctattattcgtcctttgatggcgtggttgttctttggtttgcggccgagcgcaacgaccaaggcctgtaccaaaaacgaagttgataatcagatatttgagttgtaacaagaaactaaagcattattttagcagtagcacgaatcaggatctaaaatgaacgcatccggaccaggcatcaaataaaacgaaaggctcagtcgaaagactgggcctttcgttttatctgttgtttgtcggtgaacgctctctactagagtcacactggctcaccttcgggtgggcctttctgcgtttatatagagggaaatgtgcgcggaacccctatttgtttatttttctaaatacattcaaatatgtatccgctcatgagacaataaccctgataaatgcttcaataatattgaaaaaggaagagtatgagtattcaacatttccgtgtcgcccttattcccttttttgcggcattttgccttcctgtttttgctcacccagaaacgctggtgaaagtaaaagatgctgaagatcagttgggtgcacgagtgggttacatcgaactggatctcaacagcggtaagatccttgagagttttcgccccgaagaacgttttccaatgatgagcacttttaaagttctgctatgtggcgcggtattatcccgtattgacgccgggcaagagcaactcggtcgccgcatacactattctcagaatgacttggttgagtactcaccagtcacagaaaagcatcttacggatggcatgacagtaagagaattatgcagtgctgccataaccatgagtgataacactgcggccaacttacttctgacaacgatcggaggaccgaaggagctaaccgcttttttgcacaacatgggggatcatgtaactcgccttgatcgttgggaaccggagctgaatgaagccataccaaacgacgagcgtgacaccacgatgcctgtagcaatggcaacaacgttgcgcaaactattaactggcgaactacttactctagcttcccggcaacaattaatagactggatggaggcggataaagttgcaggaccacttctgcgctcggcccttccggctggctggtttattgctgataaatctggagccggtgagcgtgggtcacgcggtatcattgcagcactggggccagatggtaagccctcccgtatcgtagttatctacacgacggggagtcaggcaactatggatgaacgaaatagacagatcgctgagataggtgcctcactgattaagcattggtaactgtcagaccaagtttactcatatatactttagattgatttaaaacttcatttttaatttaaaaggatctaggtgaagatcctttttgataatctcatgaccaaaatcccttaacgtgagttttcgttccactgagcgtcagaccccgtagaaaagatcaaaggatcttcttgagatcctttttttctgcgcgtaatctgctgcttgcaaacaaaaaaaccaccgctaccagcggtggtttgtttgccggatcaagagctaccaactctttttccgaaggtaactggcttcagcagagcgcagataccaaatactgttcttctagtgtagccgtagttaggccaccacttcaagaactctgtagcaccgcctacatacctcgctctgctaatcctgttaccagtggctgctgccagtggcgataagtcgtgtcttaccgggttggactcaagacgatagttaccggataaggcgcagcggtcgggctgaacggggggttcgtgcacacagcccagcttggagcgaacgacctacaccgaactgagatacctacagcgtgagctatgagaaagcgccacgcttcccgaagggagaaaggcggacaggtatccggtaagcggcagggtcggaacaggagagcgcacgagggagcttccagggggaaacgcctggtatctttatagtcctgtcgggtttcgccacctctgacttgagcgtcgatttttgtgatgctcgtcaggggggcggagcctatggaaaaacgccagcaacgcggcctttttacggttcctggccttttgctggccttttgctcacatgttctttcctgcgttatcccctgattctgtggataaccgtattaccgccagagaatataaaaagccagattattaatccggcttttttattatttgacgcgttttgagattcaaaattcaatctgtttggacctggataagacacaagagcgacatcctgacatgaacgccgtaaacagcaaatcctggttgaacacgtatccttttgggggcctcccgctacgacgctcgctccagctggggcttccttactatacacagcgcgcatatttcacggttgccagatgtcaagatggccaagttgaccagtgccgttccggtgctcaccgcgcgcgacgtcgccggagcggtcgagttctggaccgaccggctcgggttctcccgggacttcgtggaggacgacttcgccggtgtggtccgggacgacgtgaccctgttcatcagcgcggtccaggaccaggtggtgccggacaacaccctggcctgggtgtgggtgcgcggcctggacgagctgtacgccgagtggtcggaggtcgtgtccacgaacttccgggacgcctccgggccggccatgaccgagatcggcgagcagccgtgggggcgggagttcgccctgcgcgacccggccggcaactgcgtgcacttcgtggccgaggagcaggactgaaccttccttaaaaatttaattttcattagttgcagtcactccgctttggtttcacagtcaggaataacactagctcgtcttcaccatggatgccaatctcgcctattcatggtgtataaaagttcaacatccaaagctagaacttttggaaagagaaagaatatccgaatagggcacggcgtgccgtattgttggagtggactagcagaaagtgaggaaggcacaggatgagttttctcga

SEQ ID NO: 53 - DNA, 6277 bp, artificial
  Vector Pro7D
ttttttaccaccaagcgctcttctatctaccagtcaacactaatgataatgcacgtatatgaatgacatatttgtttttggactaaagattgacttgatctgtatcattaaaacttgtaggcggcgtggcattgagacacaggctgtatttcgccgcaaaaagcatgaagtctcgttttgaaggggcgggatcgtcctacacctgtactccgtcattgttgtgcacactaggatgtgaaagcttgtcgaaaggagtcatgtcaggactggacagagaaacaagcaaacctaacatgacgatgtctgactgtttggattctgaagggtgattacgttgcttggcttacattaattcatgtttttatttactgtcagtagacataaatagcgatttttcggtgaactaatttttttcaaagtgtttcgttgaaagcagtaggatcggacgcagagcatttacgggttcacatgaggtttgaaaggacgagcgttcccttgcgtctgacacaaatcatagatgtttcacctggcgcgacgatcttcctgacggaacgctaaatatggccactagattgccaacccatatgtatttcaatagtggaaaagcccgtcaagacctaggcccaagtatatattcggaaggacatgtccgatatatctctacaaaggatgagcggagtcacactcggtcgtagcgtctttcaaacacttgctctcttggtttcatttttatcggtcatttggtcattgagcaaaaaggccctctggtagcgtttgtaggcatcgctacggcaaatgcctgttcagcacggtcacgagccattcgctcttgttcgttgggccacttttctcggatttgtgaagagtttcagcatcagtcgtcaaaatatcaaattatattcagaggtcaacagcgcttctgccaaattgcaactctatcgaaaaaacagaacgaacatggatttccaagtacaaatcttcagttttctacttatctcggccagtgtaataattagtaggggcgacattgtcatgacacaaactcctctatcctcacctgtgacccttggacaacccgcctctatcagctgccgttcctcccaatcgctggtccattccgatggaaacacgtacttgtcttggctccaacagcgccctgggcagcccccgcggctcttgatttataaaataagtaacagatttagcggcgttccggaccggttcagtggttcgggcgcaggtaccgatttcacccttaagatctcccgcgtagaggccgaggatgtaggagtgtattactgtatgcaagcaactcaatttccccaccaatggacgttcggtcaagggactaaagttgaaattaagcgtacggttgctgcgccatccgtctttatttttccgccatctgacgaacagctcaaaagcggaacggcttctgtcgtctgtctcctgaacaatttttacccgcgagaggctaaggttcagtggaaggtcgataatgcgttgcagtcgggcaactcgcaggaatctgtgacggaacaggacagcaaggactccacatacagcttatcgtcgacattgacactgtcaaaagcggactacgagaaacacaaggtgtatgcctgcgaagttacccatcagggattgtcatcaccagtgaccaaatcatttaatcgaggtgaatgcgagggccgagggtcgctcttgacgtgcggtgacgtcgaagaaaacccgggacccatggattttcaggtccaaatattttcttttcttctgatatcagcctctgtcattataagtcggggggaagtccacctcgtggaaagcggggggggtttagtacagccgggtggcgccttgagactctcttgtgcagcctcgggattcaccttttcaaactacgatatgcattgggtgaggcaggccaccggcaagggtctggagtgggtgagtgctaatggcaccgcaggtgatacttattatccaggtagcgtcaaaggccgtttcacgattagtcgcgaaaacgctaagaattctctctatttgcagatgaattcactacgagcaggtgacacagcagtctactattgtgcgagggacgttgatattgttgcgaccatcaccgattacttcgattactggggtcaaggcactttggtaacagtttctagtgcgagtactaagggtccgagtgtatttcctttagccccttcctctaaaagcacttcaggcggaacagcagcccttggctgtttggtgaaagactacttcccggaacctgtaactgtgagctggaattctggcgcgctcactagtggagttcacacttttccagccgtgttacagtcatcgggtctttattccctgtcctccgtcgtgaccgtcccgtcgagttcactaggtacgcagacatacatttgtaacgtcaatcacaagccatcgaacacaaaggtggacaagcgtgttgaacccaagagctgcgataagacccacacctgccctccctgcccagctcccgagcttctcggcggaccttcggttttcctctttccgccgaagcccaaagatactttgatgatttcacggacgccagaagtgacatgcgtggttgttgacgtaagccatgaggatccggaagtgaaatttaactggtacgtcgatggagttgaggtccataacgccaagaccaagccccgcgaggaacaatataattccacatatcgtgtggtgtcggtacttacggtccttcatcaggactggctaaatggaaaagaatacaaatgcaaggtgtccaataaagcgctccccgctcccatcgaaaagacgatcagcaaggcgaaggggcaaccacgtgaaccgcaagtatacacgctcccgccctcccgagaagaaatgacaaaaaaccaagtctccctgacctgtttggttaaaggattttacccttcggacatcgcggtagagtgggagtccaacggacaacctgagaataactacaaaacgactcctccagtcctggactcggacggatccttcttcttgtactccaaattgacggttgacaaatcccgatggcaacaaggcaacgtttttagctgctcggtcatgcatgaagctttgcacaaccactacacacaaaaatcgttgtcgctgtcgccaggaaaataaaacccaatttactttaagactagcgcaatttttttcttacattagatgaacataaaacgacgatgaggatcactgttagggaaacgatgaactacgctgaggacttcctattattcgtcctttgatggcgtggttgttctttggtttgcggccgagcgcaacgaccaaggcctgtaccaaaaacgaagttgataatcagatatttgagttgtaacaagaaactaaagcattattttagcagtagcacgaatcaggatctaaaatgaacgcatccggaccaggcatcaaataaaacgaaaggctcagtcgaaagactgggcctttcgttttatctgttgtttgtcggtgaacgctctctactagagtcacactggctcaccttcgggtgggcctttctgcgtttatatagagggaaatgtgcgcggaacccctatttgtttatttttctaaatacattcaaatatgtatccgctcatgagacaataaccctgataaatgcttcaataatattgaaaaaggaagagtatgagtattcaacatttccgtgtcgcccttattcccttttttgcggcattttgccttcctgtttttgctcacccagaaacgctggtgaaagtaaaagatgctgaagatcagttgggtgcacgagtgggttacatcgaactggatctcaacagcggtaagatccttgagagttttcgccccgaagaacgttttccaatgatgagcacttttaaagttctgctatgtggcgcggtattatcccgtattgacgccgggcaagagcaactcggtcgccgcatacactattctcagaatgacttggttgagtactcaccagtcacagaaaagcatcttacggatggcatgacagtaagagaattatgcagtgctgccataaccatgagtgataacactgcggccaacttacttctgacaacgatcggaggaccgaaggagctaaccgcttttttgcacaacatgggggatcatgtaactcgccttgatcgttgggaaccggagctgaatgaagccataccaaacgacgagcgtgacaccacgatgcctgtagcaatggcaacaacgttgcgcaaactattaactggcgaactacttactctagcttcccggcaacaattaatagactggatggaggcggataaagttgcaggaccacttctgcgctcggcccttccggctggctggtttattgctgataaatctggagccggtgagcgtgggtcacgcggtatcattgcagcactggggccagatggtaagccctcccgtatcgtagttatctacacgacggggagtcaggcaactatggatgaacgaaatagacagatcgctgagataggtgcctcactgattaagcattggtaactgtcagaccaagtttactcatatatactttagattgatttaaaacttcatttttaatttaaaaggatctaggtgaagatcctttttgataatctcatgaccaaaatcccttaacgtgagttttcgttccactgagcgtcagaccccgtagaaaagatcaaaggatcttcttgagatcctttttttctgcgcgtaatctgctgcttgcaaacaaaaaaaccaccgctaccagcggtggtttgtttgccggatcaagagctaccaactctttttccgaaggtaactggcttcagcagagcgcagataccaaatactgttcttctagtgtagccgtagttaggccaccacttcaagaactctgtagcaccgcctacatacctcgctctgctaatcctgttaccagtggctgctgccagtggcgataagtcgtgtcttaccgggttggactcaagacgatagttaccggataaggcgcagcggtcgggctgaacggggggttcgtgcacacagcccagcttggagcgaacgacctacaccgaactgagatacctacagcgtgagctatgagaaagcgccacgcttcccgaagggagaaaggcggacaggtatccggtaagcggcagggtcggaacaggagagcgcacgagggagcttccagggggaaacgcctggtatctttatagtcctgtcgggtttcgccacctctgacttgagcgtcgatttttgtgatgctcgtcaggggggcggagcctatggaaaaacgccagcaacgcggcctttttacggttcctggccttttgctggccttttgctcacatgttctttcctgcgttatcccctgattctgtggataaccgtattaccgccagagaatataaaaagccagattattaatccggcttttttattatttgacgcgttttgagattcaaaattcaatctgtttggacctggataagacacaagagcgacatcctgacatgaacgccgtaaacagcaaatcctggttgaacacgtatccttttgggggcctcccgctacgacgctcgctccagctggggcttccttactatacacagcgcgcatatttcacggttgccagatgtcaagatggccaagttgaccagtgccgttccggtgctcaccgcgcgcgacgtcgccggagcggtcgagttctggaccgaccggctcgggttctcccgggacttcgtggaggacgacttcgccggtgtggtccgggacgacgtgaccctgttcatcagcgcggtccaggaccaggtggtgccggacaacaccctggcctgggtgtgggtgcgcggcctggacgagctgtacgccgagtggtcggaggtcgtgtccacgaacttccgggacgcctccgggccggccatgaccgagatcggcgagcagccgtgggggcgggagttcgccctgcgcgacccggccggcaactgcgtgcacttcgtggccgaggagcaggactgaaccttccttaaaaatttaattttcattagttgcagtcactccgctttggtttcacagtcaggaataacactagctcgtcttcaccatggatgccaatctcgcctattcatggtgtataaaagttcaacatccaaagctagaacttttggaaagagaaagaatatccgaatagggcacggcgtgccgtattgttggagtggactagcagaaagtgaggaaggcacaggatgagttttctcga

SEQ ID NO: 54 - DNA, 6282 bp, artificial
  Vector Pro7D+ Kozak
ttttttaccaccaagcgctcttctatctaccagtcaacactaatgataatgcacgtatatgaatgacatatttgtttttggactaaagattgacttgatctgtatcattaaaacttgtaggcggcgtggcattgagacacaggctgtatttcgccgcaaaaagcatgaagtctcgttttgaaggggcgggatcgtcctacacctgtactccgtcattgttgtgcacactaggatgtgaaagcttgtcgaaaggagtcatgtcaggactggacagagaaacaagcaaacctaacatgacgatgtctgactgtttggattctgaagggtgattacgttgcttggcttacattaattcatgtttttatttactgtcagtagacataaatagcgatttttcggtgaactaatttttttcaaagtgtttcgttgaaagcagtaggatcggacgcagagcatttacgggttcacatgaggtttgaaaggacgagcgttcccttgcgtctgacacaaatcatagatgtttcacctggcgcgacgatcttcctgacggaacgctaaatatggccactagattgccaacccatatgtatttcaatagtggaaaagcccgtcaagacctaggcccaagtatatattcggaaggacatgtccgatatatctctacaaaggatgagcggagtcacactcggtcgtagcgtctttcaaacacttgctctcttggtttcatttttatcggtcatttggtcattgagcaaaaaggccctctggtagcgtttgtaggcatcgctacggcaaatgcctgttcagcacggtcacgagccattcgctcttgttcgttgggccacttttctcggatttgtgaagagtttcagcatcagtcgtcaaaatatcaaattatattcagaggtcaacagcgcttctgccaaattgcaactctatcgaaaaaacagaacgaacccaccatggatttccaagtacaaatcttcagttttctacttatctcggccagtgtaataattagtaggggcgacattgtcatgacacaaactcctctatcctcacctgtgacccttggacaacccgcctctatcagctgccgttcctcccaatcgctggtccattccgatggaaacacgtacttgtcttggctccaacagcgccctgggcagcccccgcggctcttgatttataaaataagtaacagatttagcggcgttccggaccggttcagtggttcgggcgcaggtaccgatttcacccttaagatctcccgcgtagaggccgaggatgtaggagtgtattactgtatgcaagcaactcaatttccccaccaatggacgttcggtcaagggactaaagttgaaattaagcgtacggttgctgcgccatccgtctttatttttccgccatctgacgaacagctcaaaagcggaacggcttctgtcgtctgtctcctgaacaatttttacccgcgagaggctaaggttcagtggaaggtcgataatgcgttgcagtcgggcaactcgcaggaatctgtgacggaacaggacagcaaggactccacatacagcttatcgtcgacattgacactgtcaaaagcggactacgagaaacacaaggtgtatgcctgcgaagttacccatcagggattgtcatcaccagtgaccaaatcatttaatcgaggtgaatgcgagggccgagggtcgctcttgacgtgcggtgacgtcgaagaaaacccgggacccatggattttcaggtccaaatattttcttttcttctgatatcagcctctgtcattataagtcggggggaagtccacctcgtggaaagcggggggggtttagtacagccgggtggcgccttgagactctcttgtgcagcctcgggattcaccttttcaaactacgatatgcattgggtgaggcaggccaccggcaagggtctggagtgggtgagtgctaatggcaccgcaggtgatacttattatccaggtagcgtcaaaggccgtttcacgattagtcgcgaaaacgctaagaattctctctatttgcagatgaattcactacgagcaggtgacacagcagtctactattgtgcgagggacgttgatattgttgcgaccatcaccgattacttcgattactggggtcaaggcactttggtaacagtttctagtgcgagtactaagggtccgagtgtatttcctttagccccttcctctaaaagcacttcaggcggaacagcagcccttggctgtttggtgaaagactacttcccggaacctgtaactgtgagctggaattctggcgcgctcactagtggagttcacacttttccagccgtgttacagtcatcgggtctttattccctgtcctccgtcgtgaccgtcccgtcgagttcactaggtacgcagacatacatttgtaacgtcaatcacaagccatcgaacacaaaggtggacaagcgtgttgaacccaagagctgcgataagacccacacctgccctccctgcccagctcccgagcttctcggcggaccttcggttttcctctttccgccgaagcccaaagatactttgatgatttcacggacgccagaagtgacatgcgtggttgttgacgtaagccatgaggatccggaagtgaaatttaactggtacgtcgatggagttgaggtccataacgccaagaccaagccccgcgaggaacaatataattccacatatcgtgtggtgtcggtacttacggtccttcatcaggactggctaaatggaaaagaatacaaatgcaaggtgtccaataaagcgctccccgctcccatcgaaaagacgatcagcaaggcgaaggggcaaccacgtgaaccgcaagtatacacgctcccgccctcccgagaagaaatgacaaaaaaccaagtctccctgacctgtttggttaaaggattttacccttcggacatcgcggtagagtgggagtccaacggacaacctgagaataactacaaaacgactcctccagtcctggactcggacggatccttcttcttgtactccaaattgacggttgacaaatcccgatggcaacaaggcaacgtttttagctgctcggtcatgcatgaagctttgcacaaccactacacacaaaaatcgttgtcgctgtcgccaggaaaataaaacccaatttactttaagactagcgcaatttttttcttacattagatgaacataaaacgacgatgaggatcactgttagggaaacgatgaactacgctgaggacttcctattattcgtcctttgatggcgtggttgttctttggtttgcggccgagcgcaacgaccaaggcctgtaccaaaaacgaagttgataatcagatatttgagttgtaacaagaaactaaagcattattttagcagtagcacgaatcaggatctaaaatgaacgcatccggaccaggcatcaaataaaacgaaaggctcagtcgaaagactgggcctttcgttttatctgttgtttgtcggtgaacgctctctactagagtcacactggctcaccttcgggtgggcctttctgcgtttatatagagggaaatgtgcgcggaacccctatttgtttatttttctaaatacattcaaatatgtatccgctcatgagacaataaccctgataaatgcttcaataatattgaaaaaggaagagtatgagtattcaacatttccgtgtcgcccttattcccttttttgcggcattttgccttcctgtttttgctcacccagaaacgctggtgaaagtaaaagatgctgaagatcagttgggtgcacgagtgggttacatcgaactggatctcaacagcggtaagatccttgagagttttcgccccgaagaacgttttccaatgatgagcacttttaaagttctgctatgtggcgcggtattatcccgtattgacgccgggcaagagcaactcggtcgccgcatacactattctcagaatgacttggttgagtactcaccagtcacagaaaagcatcttacggatggcatgacagtaagagaattatgcagtgctgccataaccatgagtgataacactgcggccaacttacttctgacaacgatcggaggaccgaaggagctaaccgcttttttgcacaacatgggggatcatgtaactcgccttgatcgttgggaaccggagctgaatgaagccataccaaacgacgagcgtgacaccacgatgcctgtagcaatggcaacaacgttgcgcaaactattaactggcgaactacttactctagcttcccggcaacaattaatagactggatggaggcggataaagttgcaggaccacttctgcgctcggcccttccggctggctggtttattgctgataaatctggagccggtgagcgtgggtcacgcggtatcattgcagcactggggccagatggtaagccctcccgtatcgtagttatctacacgacggggagtcaggcaactatggatgaacgaaatagacagatcgctgagataggtgcctcactgattaagcattggtaactgtcagaccaagtttactcatatatactttagattgatttaaaacttcatttttaatttaaaaggatctaggtgaagatcctttttgataatctcatgaccaaaatcccttaacgtgagttttcgttccactgagcgtcagaccccgtagaaaagatcaaaggatcttcttgagatcctttttttctgcgcgtaatctgctgcttgcaaacaaaaaaaccaccgctaccagcggtggtttgtttgccggatcaagagctaccaactctttttccgaaggtaactggcttcagcagagcgcagataccaaatactgttcttctagtgtagccgtagttaggccaccacttcaagaactctgtagcaccgcctacatacctcgctctgctaatcctgttaccagtggctgctgccagtggcgataagtcgtgtcttaccgggttggactcaagacgatagttaccggataaggcgcagcggtcgggctgaacggggggttcgtgcacacagcccagcttggagcgaacgacctacaccgaactgagatacctacagcgtgagctatgagaaagcgccacgcttcccgaagggagaaaggcggacaggtatccggtaagcggcagggtcggaacaggagagcgcacgagggagcttccagggggaaacgcctggtatctttatagtcctgtcgggtttcgccacctctgacttgagcgtcgatttttgtgatgctcgtcaggggggcggagcctatggaaaaacgccagcaacgcggcctttttacggttcctggccttttgctggccttttgctcacatgttctttcctgcgttatcccctgattctgtggataaccgtattaccgccagagaatataaaaagccagattattaatccggcttttttattatttgacgcgttttgagattcaaaattcaatctgtttggacctggataagacacaagagcgacatcctgacatgaacgccgtaaacagcaaatcctggttgaacacgtatccttttgggggcctcccgctacgacgctcgctccagctggggcttccttactatacacagcgcgcatatttcacggttgccagatgtcaagatggccaagttgaccagtgccgttccggtgctcaccgcgcgcgacgtcgccggagcggtcgagttctggaccgaccggctcgggttctcccgggacttcgtggaggacgacttcgccggtgtggtccgggacgacgtgaccctgttcatcagcgcggtccaggaccaggtggtgccggacaacaccctggcctgggtgtgggtgcgcggcctggacgagctgtacgccgagtggtcggaggtcgtgtccacgaacttccgggacgcctccgggccggccatgaccgagatcggcgagcagccgtgggggcgggagttcgccctgcgcgacccggccggcaactgcgtgcacttcgtggccgaggagcaggactgaaccttccttaaaaatttaattttcattagttgcagtcactccgctttggtttcacagtcaggaataacactagctcgtcttcaccatggatgccaatctcgcctattcatggtgtataaaagttcaacatccaaagctagaacttttggaaagagaaagaatatccgaatagggcacggcgtgccgtattgttggagtggactagcagaaagtgaggaaggcacaggatgagttttctcga

SEQ ID NO: 55 - DNA, 5716 bp, artificial
  Vector NVB12
gagattcaaaattcaatctgtttggacctggataagacacaagagcgacatcctgacatgaacgccgtaaacagcaaatcctggttgaacacgtatccttttgggggcctcccgctacgacgctcgctccagctggggcttccttactatacacagcgcgcatatttcacggttgccagatgtcaagatggccaagttgaccagtgccgttccggtgctcaccgcgcgcgacgtcgccggagcggtcgagttctggaccgaccggctcgggttctcccgggacttcgtggaggacgacttcgccggtgtggtccgggacgacgtgaccctgttcatcagcgcggtccaggaccaggtggtgccggacaacaccctggcctgggtgtgggtgcgcggcctggacgagctgtacgccgagtggtcggaggtcgtgtccacgaacttccgggacgcctccgggccggccatgaccgagatcggcgagcagccgtgggggcgggagttcgccctgcgcgacccggccggcaactgcgtgcacttcgtggccgaggagcaggactgaaccttccttaaaaatttaattttcattagttgcagtcactccgctttggtttcacagtcaggaataacactagctcgtcttcaccatggatgccaatctcgcctattcatggtgtataaaagttcaacatccaaagctagaacttttggaaagagaaagaatatccgaatagggcacggcgtgccgtattgttggagtggactagcagaaagtgaggaaggcacaggatgagttttctcgaaagacgcatatgcggaagtgactgtaaacgagaagtgcacgaagccttttcttgtgacgtcacaaaccgaacagccctacgtggcgtgcgactttccggcactttggatatcgttgccctatatgtattgggtgtatacatgtcgtattccaactacgacagaaaacagtcagttacgggtattcgaacttccggcacctgcagcgaggagttttgtgtccgtcgcacatcctccgtgctttcggcacctacgtaggcggcaaacttcctgccttccgcccgccttgcggcattccggctccgggccagaattgcccgggtgttcacaattttgcctcctcacgaaaaaacgttctactttgtattttggtcgggtttcggatccttccagcaaccattctcattcaaagtcaccacttgtgcgaacgatctatggacttccaagtgcagatcataagctttttgttaatctctgcttccgtaattatgtcacgtggccaaattgtcttgtcgcaatcccccgcgattttatctgcatccccgggtgagaaggtgaccatgacatgcagagcatcgtcatcggtgtcatacattcactggttccaacagaagcccggtagttcgccgaaaccctggatttatgctacctctaatcttgccagtggggtaccggttcggttttcaggatcgggctcgggaaccagctattctctaactatctcacgcgttgaagcagaggacgcggctacgtactattgccagcagtggactagtaatccacccacgttcggtggaggtacgaaactcgagatcaagcgaacagtcgctgccccaagcgtttttattttcccgccttccgatgagcagttgaaatccggcaccgcgtccgttgtttgccttctcaataatttttacccaagggaagcgaaggttcaatggaaagtcgacaatgccttgcaatctggaaactcccaagaatccgtgactgaacaggatagcaaggactctacctacagtctgagcagtacactcacgctgagtaaagcggattacgagaaacataaggtctacgcctgtgaagtaacgcaccaaggcttatcctcgccggtcacgaaatcgtttaaccgaggagaatgtgagggccgagggtcgctcttgacgtgcggtgacgtcgaagaaaacccgggacccatggggtggtcactgatattgttgttccttgtggcggtggcgacacgagtattgtctcaagtacagcttcagcaacctggagccgaactagtgaagccaggggccagcgttaaaatgtcttgcaaggcctcagggtacacatttaccagctataatatgcattgggtgaagcaaacacccgggcggggcctggaatggattggtgcaatttatcccggaaacggagatacgtcttacaaccagaaatttaagggaaaagctaccttaacagccgataaatcctctagcacggcctatatgcagctgtcgtccttgacaagcgaggactccgccgtatattattgtgcacgtagcacgtattacggcggagactggtacttcaacgtttggggggcagggacaacagttacagtatcagcggcgagtaccaaaggtcccagcgtattcccgttggcgcccagctctaaatccacgagcggaggtacggctgcacttggatgtctcgtgaaggattattttcctgaacctgtaactgtcagttggaatagcggagcactaacttcaggagtgcatacctttccggcggttctccagtcctccggcctctatagtctatcctcggtagtgactgtaccctcatcctcccttggtacgcaaacgtacatttgcaatgtcaaccacaaaccgtccaatacgaaagtcgacaagaaagttgaacctaagagttgcgacaaaacccacacctgtccaccatgcccggctccagagttgctgggtggtccgtccgtgttcctctttccgccgaaaccaaaggatacactgatgatctctaggactccagaggttacttgcgtcgtcgttgatgtcagtcatgaggaccccgaggtgaagttcaattggtacgtagacggcgttgaggttcacaacgccaaaactaaaccacgagaggagcaatacaattcgacctaccgggtcgtatcggttctcaccgtgttacaccaagactggcttaatggcaaggaatacaaatgtaaggtatcaaataaggccttgccggcccccatcgaaaagactattagtaaagctaagggccagccaagggaaccacaagtgtacacattacctccatcgcgtgacgaattgactaagaatcaagtgtcattgacctgcctggtcaaaggattctacccgtcagatatcgcggtggaatgggaatcgaatggacagccggagaacaactacaaaaccacccccccggttctcgattcggacggctcgttctttctctactcgaagttgaccgtcgataaatcgcgctggcagcaaggcaacgtgttttcgtgctcggtcatgcacgaagctctgcacaaccactacacgcagaagtcgctatcgctttcgcctggcaaataaaacccaatttactttaagactagcgcaatttttttcttacattagatgaacataaaacgacgatgaggatcactgttagggaaacgatgaactacgctgaggacttcctattattcgtcctttgatggcgtggttgttctttggtttgcggccgagcgcaacgaccaaggcctgtaccaaaaacgaagttgataatcagatatttgagttgtaacaagaaactaaagcattattttagcagtagcacgaatcaggatctaaaatgaacgcatccggaccaggcatcaaataaaacgaaaggctcagtcgaaagactgggcctttcgttttatctgttgtttgtcggtgaacgctctctactagagtcacactggctcaccttcgggtgggcctttctgcgtttatatagagggaaatgtgcgcggaacccctatttgtttatttttctaaatacattcaaatatgtatccgctcatgagacaataaccctgataaatgcttcaataatattgaaaaaggaagagtatgagtattcaacatttccgtgtcgcccttattcccttttttgcggcattttgccttcctgtttttgctcacccagaaacgctggtgaaagtaaaagatgctgaagatcagttgggtgcacgagtgggttacatcgaactggatctcaacagcggtaagatccttgagagttttcgccccgaagaacgttttccaatgatgagcacttttaaagttctgctatgtggcgcggtattatcccgtattgacgccgggcaagagcaactcggtcgccgcatacactattctcagaatgacttggttgagtactcaccagtcacagaaaagcatcttacggatggcatgacagtaagagaattatgcagtgctgccataaccatgagtgataacactgcggccaacttacttctgacaacgatcggaggaccgaaggagctaaccgcttttttgcacaacatgggggatcatgtaactcgccttgatcgttgggaaccggagctgaatgaagccataccaaacgacgagcgtgacaccacgatgcctgtagcaatggcaacaacgttgcgcaaactattaactggcgaactacttactctagcttcccggcaacaattaatagactggatggaggcggataaagttgcaggaccacttctgcgctcggcccttccggctggctggtttattgctgataaatctggagccggtgagcgtgggtcacgcggtatcattgcagcactggggccagatggtaagccctcccgtatcgtagttatctacacgacggggagtcaggcaactatggatgaacgaaatagacagatcgctgagataggtgcctcactgattaagcattggtaactgtcagaccaagtttactcatatatactttagattgatttaaaacttcatttttaatttaaaaggatctaggtgaagatcctttttgataatctcatgaccaaaatcccttaacgtgagttttcgttccactgagcgtcagaccccgtagaaaagatcaaaggatcttcttgagatcctttttttctgcgcgtaatctgctgcttgcaaacaaaaaaaccaccgctaccagcggtggtttgtttgccggatcaagagctaccaactctttttccgaaggtaactggcttcagcagagcgcagataccaaatactgttcttctagtgtagccgtagttaggccaccacttcaagaactctgtagcaccgcctacatacctcgctctgctaatcctgttaccagtggctgctgccagtggcgataagtcgtgtcttaccgggttggactcaagacgatagttaccggataaggcgcagcggtcgggctgaacggggggttcgtgcacacagcccagcttggagcgaacgacctacaccgaactgagatacctacagcgtgagctatgagaaagcgccacgcttcccgaagggagaaaggcggacaggtatccggtaagcggcagggtcggaacaggagagcgcacgagggagcttccagggggaaacgcctggtatctttatagtcctgtcgggtttcgccacctctgacttgagcgtcgatttttgtgatgctcgtcaggggggcggagcctatggaaaaacgccagcaacgcggcctttttacggttcctggccttttgctggccttttgctcacatgttctttcctgcgttatcccctgattctgtggataaccgtattaccgccagagaatataaaaagccagattattaatccggcttttttattatttgacgcgtttt

SEQ ID NO: 56 - DNA, 5686 bp, artificial
  NVB13
gagattcaaaattcaatctgtttggacctggataagacacaagagcgacatcctgacatgaacgccgtaaacagcaaatcctggttgaacacgtatccttttgggggcctcccgctacgacgctcgctccagctggggcttccttactatacacagcgcgcatatttcacggttgccagatgtcaagatggccaagttgaccagtgccgttccggtgctcaccgcgcgcgacgtcgccggagcggtcgagttctggaccgaccggctcgggttctcccgggacttcgtggaggacgacttcgccggtgtggtccgggacgacgtgaccctgttcatcagcgcggtccaggaccaggtggtgccggacaacaccctggcctgggtgtgggtgcgcggcctggacgagctgtacgccgagtggtcggaggtcgtgtccacgaacttccgggacgcctccgggccggccatgaccgagatcggcgagcagccgtgggggcgggagttcgccctgcgcgacccggccggcaactgcgtgcacttcgtggccgaggagcaggactgaaccttccttaaaaatttaattttcattagttgcagtcactccgctttggtttcacagtcaggaataacactagctcgtcttcaccatggatgccaatctcgcctattcatggtgtataaaagttcaacatccaaagctagaacttttggaaagagaaagaatatccgaatagggcacggcgtgccgtattgttggagtggactagcagaaagtgaggaaggcacaggatgagttttctcgattttcatatgcggaagtgactgtaaacgagaagtgcacgaagccttttcttgtgacgtcacaaaccgaacagccctacgtggcgtgcgactttccggcactttggatatcgttgccctatatgtattgggtgtatacatgtcgtattccaactacgacagaaaacagtcagttacgggtattcgaacttccggcacctgcagcgaggagttttgtgtccgtcgcacatcctccgtgctttcggcacctacgtaggcggcaaacttcctgccttccgcccgccttgcggcattccggctccgggccagaattgcccgggtgttcacaattttgcctcctcacgaaaaaacgttctactttgtattttggtcgggtttcggatccttccagcaaccattctcattcaaagtcaccacttgtgcgaacgatctatggacttccaagtgcagatcataagctttttgttaatctctgcttccgtaattatgtcacgtggccaaattgtcttgtcgcaatcccccgcgattttatctgcatccccgggtgagaaggtgaccatgacatgcagagcatcgtcatcggtgtcatacattcactggttccaacagaagcccggtagttcgccgaaaccctggatttatgctacctctaatcttgccagtggggtaccggttcggttttcaggatcgggctcgggaaccagctattctctaactatctcacgcgttgaagcagaggacgcggctacgtactattgccagcagtggactagtaatccacccacgttcggtggaggtacgaaactcgagatcaagcgaacagtcgctgccccaagcgtttttattttcccgccttccgatgagcagttgaaatccggcaccgcgtccgttgtttgccttctcaataatttttacccaagggaagcgaaggttcaatggaaagtcgacaatgccttgcaatctggaaactcccaagaatccgtgactgaacaggatagcaaggactctacctacagtctgagcagtacactcacgctgagtaaagcggattacgagaaacataaggtctacgcctgtgaagtaacgcaccaaggcttatcctcgccggtcacgaaatcgtttaaccgaggagaatgtgagggccgagggtcgctcttgacgtgcggtgacgtcgaagaaaacccgggacccatggggtggtcactgatattgttgttccttgtggcggtggcgacacgagtattgtctcaagtacagcttcagcaacctggagccgaactagtgaagccaggggccagcgttaaaatgtcttgcaaggcctcagggtacacatttaccagctataatatgcattgggtgaagcaaacacccgggcggggcctggaatggattggtgcaatttatcccggaaacggagatacgtcttacaaccagaaatttaagggaaaagctaccttaacagccgataaatcctctagcacggcctatatgcagctgtcgtccttgacaagcgaggactccgccgtatattattgtgcacgtagcacgtattacggcggagactggtacttcaacgtttggggggcagggacaacagttacagtatcagcggcgagtaccaaaggtcccagcgtattcccgttggcgcccagctctaaatccacgagcggaggtacggctgcacttggatgtctcgtgaaggattattttcctgaacctgtaactgtcagttggaatagcggagcactaacttcaggagtgcatacctttccggcggttctccagtcctccggcctctatagtctatcctcggtagtgactgtaccctcatcctcccttggtacgcaaacgtacatttgcaatgtcaaccacaaaccgtccaatacgaaagtcgacaagaaagttgaacctaagagttgcgacaaaacccacacctgtccaccatgcccggctccagagttgctgggtggtccgtccgtgttcctctttccgccgaaaccaaaggatacactgatgatctctaggactccagaggttacttgcgtcgtcgttgatgtcagtcatgaggaccccgaggtgaagttcaattggtacgtagacggcgttgaggttcacaacgccaaaactaaaccacgagaggagcaatacaattcgacctaccgggtcgtatcggttctcaccgtgttacaccaagactggcttaatggcaaggaatacaaatgtaaggtatcaaataaggccttgccggcccccatcgaaaagactattagtaaagctaagggccagccaagggaaccacaagtgtacacattacctccatcgcgtgacgaattgactaagaatcaagtgtcattgacctgcctggtcaaaggattctacccgtcagatatcgcggtggaatgggaatcgaatggacagccggagaacaactacaaaaccacccccccggttctcgattcggacggctcgttctttctctactcgaagttgaccgtcgataaatcgcgctggcagcaaggcaacgtgttttcgtgctcggtcatgcacgaagctctgcacaaccactacacgcagaagtcgctatcgctttcgcctggcaaataaaaccaccttccttaaaaatttaattttcattagttgcagtcactccgctttggtttcacagtcaggaataacactagctcgtcttcaccatggatgccaatctcgcctattcatggtgtataaaagttcaacatccaaagctagaacttttggaaagagaaagaatatccgaatagggcacggcgtgccgtattgttggagtggactagcagaaagtgaggaaggcacaggatgagttttctcgagagcccaggcatcaaataaaacgaaaggctcagtcgaaagactgggcctttcgttttatctgttgtttgtcggtgaacgctctctactagagtcacactggctcaccttcgggtgggcctttctgcgtttatatagagggaaatgtgcgcggaacccctatttgtttatttttctaaatacattcaaatatgtatccgctcatgagacaataaccctgataaatgcttcaataatattgaaaaaggaagagtatgagtattcaacatttccgtgtcgcccttattcccttttttgcggcattttgccttcctgtttttgctcacccagaaacgctggtgaaagtaaaagatgctgaagatcagttgggtgcacgagtgggttacatcgaactggatctcaacagcggtaagatccttgagagttttcgccccgaagaacgttttccaatgatgagcacttttaaagttctgctatgtggcgcggtattatcccgtattgacgccgggcaagagcaactcggtcgccgcatacactattctcagaatgacttggttgagtactcaccagtcacagaaaagcatcttacggatggcatgacagtaagagaattatgcagtgctgccataaccatgagtgataacactgcggccaacttacttctgacaacgatcggaggaccgaaggagctaaccgcttttttgcacaacatgggggatcatgtaactcgccttgatcgttgggaaccggagctgaatgaagccataccaaacgacgagcgtgacaccacgatgcctgtagcaatggcaacaacgttgcgcaaactattaactggcgaactacttactctagcttcccggcaacaattaatagactggatggaggcggataaagttgcaggaccacttctgcgctcggcccttccggctggctggtttattgctgataaatctggagccggtgagcgtgggtcacgcggtatcattgcagcactggggccagatggtaagccctcccgtatcgtagttatctacacgacggggagtcaggcaactatggatgaacgaaatagacagatcgctgagataggtgcctcactgattaagcattggtaactgtcagaccaagtttactcatatatactttagattgatttaaaacttcatttttaatttaaaaggatctaggtgaagatcctttttgataatctcatgaccaaaatcccttaacgtgagttttcgttccactgagcgtcagaccccgtagaaaagatcaaaggatcttcttgagatcctttttttctgcgcgtaatctgctgcttgcaaacaaaaaaaccaccgctaccagcggtggtttgtttgccggatcaagagctaccaactctttttccgaaggtaactggcttcagcagagcgcagataccaaatactgttcttctagtgtagccgtagttaggccaccacttcaagaactctgtagcaccgcctacatacctcgctctgctaatcctgttaccagtggctgctgccagtggcgataagtcgtgtcttaccgggttggactcaagacgatagttaccggataaggcgcagcggtcgggctgaacggggggttcgtgcacacagcccagcttggagcgaacgacctacaccgaactgagatacctacagcgtgagctatgagaaagcgccacgcttcccgaagggagaaaggcggacaggtatccggtaagcggcagggtcggaacaggagagcgcacgagggagcttccagggggaaacgcctggtatctttatagtcctgtcgggtttcgccacctctgacttgagcgtcgatttttgtgatgctcgtcaggggggcggagcctatggaaaaacgccagcaacgcggcctttttacggttcctggccttttgctggccttttgctcacatgttctttcctgcgttatcccctgattctgtggataaccgtattaccgccagagaatataaaaagccagattattaatccggcttttttattatttgacgcgtttt

SEQ ID NO: 57 - DNA, 5716 bp, artificial
  NVB14
gagattcaaaattcaatctgtttggacctggataagacacaagagcgacatcctgacatgaacgccgtaaacagcaaatcctggttgaacacgtatccttttgggggcctcccgctacgacgctcgctccagctggggcttccttactatacacagcgcgcatatttcacggttgccagatgtcaagatggccaagttgaccagtgccgttccggtgctcaccgcgcgcgacgtcgccggagcggtcgagttctggaccgaccggctcgggttctcccgggacttcgtggaggacgacttcgccggtgtggtccgggacgacgtgaccctgttcatcagcgcggtccaggaccaggtggtgccggacaacaccctggcctgggtgtgggtgcgcggcctggacgagctgtacgccgagtggtcggaggtcgtgtccacgaacttccgggacgcctccgggccggccatgaccgagatcggcgagcagccgtgggggcgggagttcgccctgcgcgacccggccggcaactgcgtgcacttcgtggccgaggagcaggactgaaccttccttaaaaatttaattttcattagttgcagtcactccgctttggtttcacagtcaggaataacactagctcgtcttcaccatggatgccaatctcgcctattcatggtgtataaaagttcaacatccaaagctagaacttttggaaagagaaagaatatccgaatagggcacggcgtgccgtattgttggagtggactagcagaaagtgaggaaggcacaggatgagttttctcgaaagacgcatatgcggaagtgactgtaaacgagaagtgcacgaagccttttcttgtgacgtcacaaaccgaacagccctacgtggcgtgcgactttccggcactttggatatcgttgccctatatgtattgggtgtatacatgtcgtattccaactacgacagaaaacagtcagttacgggtattcgaacttccggcacctgcagcgaggagttttgtgtccgtcgcacatcctccgtgctttcggcacctacgtaggcggcaaacttcctgccttccgcccgccttgcggcattccggctccgggccagaattgcccgggtgttcacaattttgcctcctcacgaaaaaacgttctactttgtattttggtcgggtttcggatccttccagcaaccattctcattcaaagtcaccacttgtgcgaacgatctatggacatgcgagtcccggctcaacttctcggattactactgttgtggttgtcgggtgcccgctgccaaattgtcttgtcgcaatcccccgcgattttatctgcatccccgggtgagaaggtgaccatgacatgcagagcatcgtcatcggtgtcatacattcactggttccaacagaagcccggtagttcgccgaaaccctggatttatgctacctctaatcttgccagtggggtaccggttcggttttcaggatcgggctcgggaaccagctattctctaactatctcacgcgttgaagcagaggacgcggctacgtactattgccagcagtggactagtaatccacccacgttcggtggaggtacgaaactcgagatcaagcgaacagtcgctgccccaagcgtttttattttcccgccttccgatgagcagttgaaatccggcaccgcgtccgttgtttgccttctcaataatttttacccaagggaagcgaaggttcaatggaaagtcgacaatgccttgcaatctggaaactcccaagaatccgtgactgaacaggatagcaaggactctacctacagtctgagcagtacactcacgctgagtaaagcggattacgagaaacataaggtctacgcctgtgaagtaacgcaccaaggcttatcctcgccggtcacgaaatcgtttaaccgaggagaatgtgagggccgagggtcgctcttgacgtgcggtgacgtcgaagaaaacccgggacccatggagtttgggctgtcatgggtattcctcgttgccctgttccgaggtgtgcagtgccaagtacagcttcagcaacctggagccgaactagtgaagccaggggccagcgttaaaatgtcttgcaaggcctcagggtacacatttaccagctataatatgcattgggtgaagcaaacacccgggcggggcctggaatggattggtgcaatttatcccggaaacggagatacgtcttacaaccagaaatttaagggaaaagctaccttaacagccgataaatcctctagcacggcctatatgcagctgtcgtccttgacaagcgaggactccgccgtatattattgtgcacgtagcacgtattacggcggagactggtacttcaacgtttggggggcagggacaacagttacagtatcagcggcgagtaccaaaggtcccagcgtattcccgttggcgcccagctctaaatccacgagcggaggtacggctgcacttggatgtctcgtgaaggattattttcctgaacctgtaactgtcagttggaatagcggagcactaacttcaggagtgcatacctttccggcggttctccagtcctccggcctctatagtctatcctcggtagtgactgtaccctcatcctcccttggtacgcaaacgtacatttgcaatgtcaaccacaaaccgtccaatacgaaagtcgacaagaaagttgaacctaagagttgcgacaaaacccacacctgtccaccatgcccggctccagagttgctgggtggtccgtccgtgttcctctttccgccgaaaccaaaggatacactgatgatctctaggactccagaggttacttgcgtcgtcgttgatgtcagtcatgaggaccccgaggtgaagttcaattggtacgtagacggcgttgaggttcacaacgccaaaactaaaccacgagaggagcaatacaattcgacctaccgggtcgtatcggttctcaccgtgttacaccaagactggcttaatggcaaggaatacaaatgtaaggtatcaaataaggccttgccggcccccatcgaaaagactattagtaaagctaagggccagccaagggaaccacaagtgtacacattacctccatcgcgtgacgaattgactaagaatcaagtgtcattgacctgcctggtcaaaggattctacccgtcagatatcgcggtggaatgggaatcgaatggacagccggagaacaactacaaaaccacccccccggttctcgattcggacggctcgttctttctctactcgaagttgaccgtcgataaatcgcgctggcagcaaggcaacgtgttttcgtgctcggtcatgcacgaagctctgcacaaccactacacgcagaagtcgctatcgctttcgcctggcaaataaaacccaatttactttaagactagcgcaatttttttcttacattagatgaacataaaacgacgatgaggatcactgttagggaaacgatgaactacgctgaggacttcctattattcgtcctttgatggcgtggttgttctttggtttgcggccgagcgcaacgaccaaggcctgtaccaaaaacgaagttgataatcagatatttgagttgtaacaagaaactaaagcattattttagcagtagcacgaatcaggatctaaaatgaacgcatccggaccaggcatcaaataaaacgaaaggctcagtcgaaagactgggcctttcgttttatctgttgtttgtcggtgaacgctctctactagagtcacactggctcaccttcgggtgggcctttctgcgtttatatagagggaaatgtgcgcggaacccctatttgtttatttttctaaatacattcaaatatgtatccgctcatgagacaataaccctgataaatgcttcaataatattgaaaaaggaagagtatgagtattcaacatttccgtgtcgcccttattcccttttttgcggcattttgccttcctgtttttgctcacccagaaacgctggtgaaagtaaaagatgctgaagatcagttgggtgcacgagtgggttacatcgaactggatctcaacagcggtaagatccttgagagttttcgccccgaagaacgttttccaatgatgagcacttttaaagttctgctatgtggcgcggtattatcccgtattgacgccgggcaagagcaactcggtcgccgcatacactattctcagaatgacttggttgagtactcaccagtcacagaaaagcatcttacggatggcatgacagtaagagaattatgcagtgctgccataaccatgagtgataacactgcggccaacttacttctgacaacgatcggaggaccgaaggagctaaccgcttttttgcacaacatgggggatcatgtaactcgccttgatcgttgggaaccggagctgaatgaagccataccaaacgacgagcgtgacaccacgatgcctgtagcaatggcaacaacgttgcgcaaactattaactggcgaactacttactctagcttcccggcaacaattaatagactggatggaggcggataaagttgcaggaccacttctgcgctcggcccttccggctggctggtttattgctgataaatctggagccggtgagcgtgggtcacgcggtatcattgcagcactggggccagatggtaagccctcccgtatcgtagttatctacacgacggggagtcaggcaactatggatgaacgaaatagacagatcgctgagataggtgcctcactgattaagcattggtaactgtcagaccaagtttactcatatatactttagattgatttaaaacttcatttttaatttaaaaggatctaggtgaagatcctttttgataatctcatgaccaaaatcccttaacgtgagttttcgttccactgagcgtcagaccccgtagaaaagatcaaaggatcttcttgagatcctttttttctgcgcgtaatctgctgcttgcaaacaaaaaaaccaccgctaccagcggtggtttgtttgccggatcaagagctaccaactctttttccgaaggtaactggcttcagcagagcgcagataccaaatactgttcttctagtgtagccgtagttaggccaccacttcaagaactctgtagcaccgcctacatacctcgctctgctaatcctgttaccagtggctgctgccagtggcgataagtcgtgtcttaccgggttggactcaagacgatagttaccggataaggcgcagcggtcgggctgaacggggggttcgtgcacacagcccagcttggagcgaacgacctacaccgaactgagatacctacagcgtgagctatgagaaagcgccacgcttcccgaagggagaaaggcggacaggtatccggtaagcggcagggtcggaacaggagagcgcacgagggagcttccagggggaaacgcctggtatctttatagtcctgtcgggtttcgccacctctgacttgagcgtcgatttttgtgatgctcgtcaggggggcggagcctatggaaaaacgccagcaacgcggcctttttacggttcctggccttttgctggccttttgctcacatgttctttcctgcgttatcccctgattctgtggataaccgtattaccgccagagaatataaaaagccagattattaatccggcttttttattatttgacgcgtttt

SEQ ID NO: 58 - DNA, 5705 bp, artificial
  Vector NVB16
gagattcaaaattcaatctgtttggacctggataagacacaagagcgacatcctgacatgaacgccgtaaacagcaaatcctggttgaacacgtatccttttgggggcctcccgctacgacgctcgctccagctggggcttccttactatacacagcgcgcatatttcacggttgccagatgtcaagatggccaagttgaccagtgccgttccggtgctcaccgcgcgcgacgtcgccggagcggtcgagttctggaccgaccggctcgggttctcccgggacttcgtggaggacgacttcgccggtgtggtccgggacgacgtgaccctgttcatcagcgcggtccaggaccaggtggtgccggacaacaccctggcctgggtgtgggtgcgcggcctggacgagctgtacgccgagtggtcggaggtcgtgtccacgaacttccgggacgcctccgggccggccatgaccgagatcggcgagcagccgtgggggcgggagttcgccctgcgcgacccggccggcaactgcgtgcacttcgtggccgaggagcaggactgaaccttccttaaaaatttaattttcattagttgcagtcactccgctttggtttcacagtcaggaataacactagctcgtcttcaccatggatgccaatctcgcctattcatggtgtataaaagttcaacatccaaagctagaacttttggaaagagaaagaatatccgaatagggcacggcgtgccgtattgttggagtggactagcagaaagtgaggaaggcacaggatgagttttctcgattttcatatgcggaagtgactgtaaacgagaagtgcacgaagccttttcttgtgacgtcacaaaccgaacagccctacgtggcgtgcgactttccggcactttggatatcgttgccctatatgtattgggtgtatacatgtcgtattccaactacgacagaaaacagtcagttacgggtattcgaacttccggcacctgcagcgaggagttttgtgtccgtcgcacatcctccgtgctttcggcacctacgtaggcggcaaacttcctgccttccgcccgccttgcggcattccggctccgggccagaattgcccgggtgttcacaattttgcctcctcacgaaaaaacgttctactttgtattttggtcgggtttcggatccttccagcaaccattctcattcaaagtcaccacttgtgcgaacgtatcatgacccgactcacggtcctagcccttttggctggactgttggcgtcgtcccgcgcacaaattgtcttgtcgcaatcccccgcgattttatctgcatccccgggtgagaaggtgaccatgacatgcagagcatcgtcatcggtgtcatacattcactggttccaacagaagcccggtagttcgccgaaaccctggatttatgctacctctaatcttgccagtggggtaccggttcggttttcaggatcgggctcgggaaccagctattctctaactatctcacgcgttgaagcagaggacgcggctacgtactattgccagcagtggactagtaatccacccacgttcggtggaggtacgaaactcgagatcaagcgaacagtcgctgccccaagcgtttttattttcccgccttccgatgagcagttgaaatccggcaccgcgtccgttgtttgccttctcaataatttttacccaagggaagcgaaggttcaatggaaagtcgacaatgccttgcaatctggaaactcccaagaatccgtgactgaacaggatagcaaggactctacctacagtctgagcagtacactcacgctgagtaaagcggattacgagaaacataaggtctacgcctgtgaagtaacgcaccaaggcttatcctcgccggtcacgaaatcgtttaaccgaggagaatgtgagggccgagggtcgctcttgacgtgcggtgacgtcgaagaaaacccgggacccatgacccgactcacggtcctagcccttttggctggactgttggcgtcgtcccgcgcacaagtacagcttcagcaacctggagccgaactagtgaagccaggggccagcgttaaaatgtcttgcaaggcctcagggtacacatttaccagctataatatgcattgggtgaagcaaacacccgggcggggcctggaatggattggtgcaatttatcccggaaacggagatacgtcttacaaccagaaatttaagggaaaagctaccttaacagccgataaatcctctagcacggcctatatgcagctgtcgtccttgacaagcgaggactccgccgtatattattgtgcacgtagcacgtattacggcggagactggtacttcaacgtttggggggcagggacaacagttacagtatcagcggcgagtaccaaaggtcccagcgtattcccgttggcgcccagctctaaatccacgagcggaggtacggctgcacttggatgtctcgtgaaggattattttcctgaacctgtaactgtcagttggaatagcggagcactaacttcaggagtgcatacctttccggcggttctccagtcctccggcctctatagtctatcctcggtagtgactgtaccctcatcctcccttggtacgcaaacgtacatttgcaatgtcaaccacaaaccgtccaatacgaaagtcgacaagaaagttgaacctaagagttgcgacaaaacccacacctgtccaccatgcccggctccagagttgctgggtggtccgtccgtgttcctctttccgccgaaaccaaaggatacactgatgatctctaggactccagaggttacttgcgtcgtcgttgatgtcagtcatgaggaccccgaggtgaagttcaattggtacgtagacggcgttgaggttcacaacgccaaaactaaaccacgagaggagcaatacaattcgacctaccgggtcgtatcggttctcaccgtgttacaccaagactggcttaatggcaaggaatacaaatgtaaggtatcaaataaggccttgccggcccccatcgaaaagactattagtaaagctaagggccagccaagggaaccacaagtgtacacattacctccatcgcgtgacgaattgactaagaatcaagtgtcattgacctgcctggtcaaaggattctacccgtcagatatcgcggtggaatgggaatcgaatggacagccggagaacaactacaaaaccacccccccggttctcgattcggacggctcgttctttctctactcgaagttgaccgtcgataaatcgcgctggcagcaaggcaacgtgttttcgtgctcggtcatgcacgaagctctgcacaaccactacacgcagaagtcgctatcgctttcgcctggcaaataaaacccaatttactttaagactagcgcaatttttttcttacattagatgaacataaaacgacgatgaggatcactgttagggaaacgatgaactacgctgaggacttcctattattcgtcctttgatggcgtggttgttctttggtttgcggccgagcgcaacgaccaaggcctgtaccaaaaacgaagttgataatcagatatttgagttgtaacaagaaactaaagcattattttagcagtagcacgaatcaggatctaaaatgaacgcatccggaccaggcatcaaataaaacgaaaggctcagtcgaaagactgggcctttcgttttatctgttgtttgtcggtgaacgctctctactagagtcacactggctcaccttcgggtgggcctttctgcgtttatatagagggaaatgtgcgcggaacccctatttgtttatttttctaaatacattcaaatatgtatccgctcatgagacaataaccctgataaatgcttcaataatattgaaaaaggaagagtatgagtattcaacatttccgtgtcgcccttattcccttttttgcggcattttgccttcctgtttttgctcacccagaaacgctggtgaaagtaaaagatgctgaagatcagttgggtgcacgagtgggttacatcgaactggatctcaacagcggtaagatccttgagagttttcgccccgaagaacgttttccaatgatgagcacttttaaagttctgctatgtggcgcggtattatcccgtattgacgccgggcaagagcaactcggtcgccgcatacactattctcagaatgacttggttgagtactcaccagtcacagaaaagcatcttacggatggcatgacagtaagagaattatgcagtgctgccataaccatgagtgataacactgcggccaacttacttctgacaacgatcggaggaccgaaggagctaaccgcttttttgcacaacatgggggatcatgtaactcgccttgatcgttgggaaccggagctgaatgaagccataccaaacgacgagcgtgacaccacgatgcctgtagcaatggcaacaacgttgcgcaaactattaactggcgaactacttactctagcttcccggcaacaattaatagactggatggaggcggataaagttgcaggaccacttctgcgctcggcccttccggctggctggtttattgctgataaatctggagccggtgagcgtgggtcacgcggtatcattgcagcactggggccagatggtaagccctcccgtatcgtagttatctacacgacggggagtcaggcaactatggatgaacgaaatagacagatcgctgagataggtgcctcactgattaagcattggtaactgtcagaccaagtttactcatatatactttagattgatttaaaacttcatttttaatttaaaaggatctaggtgaagatcctttttgataatctcatgaccaaaatcccttaacgtgagttttcgttccactgagcgtcagaccccgtagaaaagatcaaaggatcttcttgagatcctttttttctgcgcgtaatctgctgcttgcaaacaaaaaaaccaccgctaccagcggtggtttgtttgccggatcaagagctaccaactctttttccgaaggtaactggcttcagcagagcgcagataccaaatactgttcttctagtgtagccgtagttaggccaccacttcaagaactctgtagcaccgcctacatacctcgctctgctaatcctgttaccagtggctgctgccagtggcgataagtcgtgtcttaccgggttggactcaagacgatagttaccggataaggcgcagcggtcgggctgaacggggggttcgtgcacacagcccagcttggagcgaacgacctacaccgaactgagatacctacagcgtgagctatgagaaagcgccacgcttcccgaagggagaaaggcggacaggtatccggtaagcggcagggtcggaacaggagagcgcacgagggagcttccagggggaaacgcctggtatctttatagtcctgtcgggtttcgccacctctgacttgagcgtcgatttttgtgatgctcgtcaggggggcggagcctatggaaaaacgccagcaacgcggcctttttacggttcctggccttttgctggccttttgctcacatgttctttcctgcgttatcccctgattctgtggataaccgtattaccgccagagaatataaaaagccagattattaatccggcttttttattatttgacgcgtttt

SEQ ID NO: 59 - DNA, 500 bp, artificial
  Termination sequence of Phatr3_J37038 (500 pb after STOP codon)
atttcagattaagttttgaacaatttgcttttattatgttgtgcaggcacgattgaaactgtgaacggtttgtgttgtatgcgtgctcactgtcaatttacggtggtttatcaggaatcggatcaggattggcaaaggtcaaaccctaccttgcccacctctaagattctaatcatcaatcaacatttgctttggagatttggctgctggaatcagccaaactgtattgggtacgagccattgccagaccagaaatagcgacccatataagctctctgccagcaaatggaaggctatctttcttaccaatttctttccccgagcggtagcggatacgaagaccgtatcaaatatatatacttacatttcaataaaggcgtccagtgacgataatggtatactgcgtatcttgtctcacgatgtagtgcgtgcaatagttagaaaaaatgtgcaagtgatccataccttgcaatttttttgggaccgagggacttttttgg

SEQ ID NO: 60 - DNA, 500 bp, artificial
  Termination sequence of Phatr3_Jdraft1443 (500 pb after STOP codon)
gtagatggtacaaacaatatgtatagtagctcttttctgtgaaagttgtattcctctcttcctttctcacagaaggacgacttgatcttccatgcgagaaaatgggctatgcactggttgttcgatggcatctccatcccgtgagcctctccacttttcgttagacaataaactcatcacacaaattagtatgacaagctgctctttaaaatcaatctcattgatcagtccgtattggatttgggaattatcttggcataccggtagttctagacaaagaaaggcaaggactatacttacttaaagtcacgtaaagatccagtcagaacggggatcgagccttgatagagagacaatcttcgccagctataaaatatgtactatccgatgtgtgtccccttgtcctttctgaaatgactcttttgtccgaatgtgcctctgactattagcaagaagctcccaaggggtaatctaccattttcaagctcgaaaaaattgga

SEQ ID NO: 61 - DNA, 175 bp, artificial
  Termination sequence of Phatr3_J35102 (175 pb after STOP codon)
cgcttattatattgcagatcatggttgttcatgttcggagcatgggctgctgtaacaacaaccctgaaacatgatcacattctgcgtgacgtcgaaaaaagagagcgcggctggtgaaatgtatgcccttttgttacagcgtagtattacaaaaaaaaaggaaaatttactgtta

SEQ ID NO: 62 - DNA, 500 bp, artificial
  Termination sequence of Phatr3_J50252 (500 pb after codon STOP)
atggaattcgatcatggaaaatggaacctaaagtgtgacctgatgtagatgatttgcgaataactctaaatcggcaaagagcttacaattaatctttaaatacgtcgtctgtcaagatataagtgaatatgcttgatataccttaaatgtgacgaggtcaaacgacgtgatttggggatagcgctccgtggttcaattccatggcacgttaattttgacagtcgtcaatcaaaactcgctattagaccaagataggaaatctatgctttgtcgtaacgaccaatagctgtggtgctgatctacgaaccaaaaaaagctgttagacctggaattgctcgtcggctatgcaagaaaattgagcttgcattttacaaatgggaaacggaacggctactcccatgggaaatcggcgacaatcccgatcctctcacaaaatgactcggaatccatgaattgtaaaaccttaagctataaagactgattcctgatttaatgaatta

SEQ ID NO: 63 - DNA, 229 bp, artificial
  Termination sequence of Phatr3_J34085 (229 pb after STOP codon)
actcctttggctctttcaacagtatgtaacgaccatcatctgatggtaaacttggaaattattgaattagtctaattatatttgcatatcgttcagtgtaagtcagttgtgccatagttcattcaacggcgtgtacgtgcgtcaaggaggtcgtgaaatttaggtttctcgaaaactccgaagcaagatgaaggtgcaaacgtcgatggaatacactgtcaacaatcgc

SEQ ID NO: 64 - DNA, 114 bp, artificial
  Termination sequence of Phatr3_J48164 (114 pb after STOP codon)
tcggaacatagtgctggtcttgttcggtcacagcagcatataggtaaaccttaaaagtgtcggaatttatacagtgtagactgtctaattagtacaagaggcttagtaccatat

SEQ ID NO: 65 - DNA, 500 bp, artificial
  Termination sequence of Phatr3_EG02422 (500 pb after STOP codon)
atggagcgaggcaattcctcctccattttattggtgctgttatattctaaaagtatttgttacatttcagttgcatcgtatcgaggtagaattgtggagagatgtgttttgatttgtagaatgaccggccttgcagttaactccaagatgcaacacagcctatgcgagatgtcgatcgacatccaggttgggcaaataaatatcgcaagatgacagacggacagaatctcggcgaaagacgttcgttcactttttcgaagtactctccagcgtcatgcggctcgtgtaaaacgaaaggaattggcaatctattcgtcatgaaattaccgctgcgcctaagatgccttgggctctttctttcgttcctcccctcgtttccatgggtcaccccgtacggtgtcaaaacttcgctccgtcttccaatttgttcgaaaatttgtcctcgacttcagtccgttacacttcggggtgatcggatagttttgctctcagaatcccgc

SEQ ID NO: 66 - DNA, 148 bp, artificial
  Termination sequence of Phatr3_J42538 (148 pb after STOP codon)
ttgtggagcgtctcattacgggtcagcgagggattatattaggtagtcgatgttttgcatataaagaatacggcgagacgaagccatttttttgcttacaacaataccttcagaaacctagagatgcttgcagtcaggattgactacc

SEQ ID NO: 67 - DNA, 351 bp, artificial
  Termination sequence of Phatr3_J48356 (351 pb after STOP codon)
ttgctcacagtcaacgatgaatccttcacgatgagaggctcacgttagcgttgcggggttcaagattggacgatgaggtggttgatccgaacggaagggtgacgagattggccctggactccgtcggtcaaagaaaaacaattgcccatcgcatagtagacacaaattcatagtatttcaaagaagaatcaactgtctatatattgttagattgactttgtcgcatttaacaccaaaaaatatgttataatgtcttaaagaacggtaaagagcaggcaataaggtagttcctatttcaaaatggtactcgaggtgtagcgatcaagcttttgttctcacgtcaaaagtaga

SEQ ID NO: 68 - DNA, 20 bp, artificial
  Primer TRA-F
cgataatgcgttgcagtcgg

SEQ ID NO: 69 - DNA, 20 bp, artificial
  Primer TRA-R
tcggacccttagtactcgca

SEQ ID NO: 70 - DNA, 20 bp, artificial
  Primer RTX-F
atctcacgcgttgaagcaga

SEQ ID NO: 71 - DNA, 20 bp, artificial
  Primer RTX-R
ccctggcttcactagttcgg

SEQ ID NO: 72 - DNA, 21 bp, artificial
  Primer HC trastuzumab - F
ctgtcattataagtcgggggg

SEQ ID NO: 73 - DNA, 21 bp, artificial
  Primer HC trastuzumab - R
tcgcgactaatcgtgaaacgg

SEQ ID NO: 74 - DNA, 21 bp, artificial
  Primer LC trastuzumab - F
aaactcctctatcctcacctg

SEQ ID NO: 75 - DNA, 20 bp, artificial
  Primer LC trastuzumab - R
caactttagtcccttgaccg

SEQ ID NO: 76 - DNA, 22 bp, artificial
  Single primer trastuzumab - F
cagcaaggactccacatacagc

SEQ ID NO: 77 - DNA, 21 bp, artificial
  Single primer trastuzumab - R
tcgcgactaatcgtgaaacgg

SEQ ID NO: 78 - DNA, 66 bp, artificial
  Primer 1 TU from pPhaNR-eGFP
gctctagatagttggaatggtacgtaccaactccataaggatccatggtgagcaagggcgaggagc

SEQ ID NO: 79 - DNA, 41 bp, artificial
  Primer 2 TU from pPhaNR-eGFP
acatgcatgctccggatgcgttcattttagatcctgatccg

SEQ ID NO: 80 - DNA, 20 bp, artificial
  Primer eGFP - F
atcatggccgacaagcagaa

SEQ ID NO: 81 - DNA, 20 bp, artificial
  Primer eGFP - R
gactgggtgctcaggtagtg

SEQ ID NO: 82 - protein, 17 aa, artificial
  Signal peptide sequence putative PDI Phaeodactylum
MKFTAAITLAFAASVSA

SEQ ID NO: 83 - DNA, 499 bp, artificial
  Sequence of Promotor HASP1
catacagtgaatgtaactttcgaattgacagtattagtagtcgtattgacagtgaggcacgcccctcaatgtgcgaggtggaaaatataccagcatgacaatgaatcttggagattcttttgctgtcatcaagattcaccgccaaatcttcaggaacctatcacgtccacaggcgatgttaattcttgagtcgtcaaaacaaagtcctgtcctacctgtagaagttgacagcgagcaattgtatgcaaacttctgactttgttataataacattaaaggtaattaagtatcttcaattaggcattttgtcactgtcagtccgttccgacaatataggtagatttggaatgaatcttttctatgctgctgcgaatcttgtacacctttgaggccgtagattctgtccgacgaagcgataattattgcaaaatacatggactcattattttgattcgatttctttttggtatccgactcgaaaagatccatcacggcgagc

SEQ ID NO: 84 - DNA, 600 bp, artificial
  Sequence of Promotor 40SRPS8
ccctgcgatagaccttttccaaactcacgcagtccaagaaaacaaaggggtgagaagtatacgcacctttcggtttcggcataattcttaaactcttgtggtcactttcttgtgaagaagctaggggcactcgttttccctcagagcctgcaaacacaaaattcctgcagtcaattgtcccaacactcggcaaaccgtatgcgcaagcaacgatgcgcagaaggccgtggatggatggcgactcgcgatatggcttcttgggtcgccagtgtggtacgtccggcgtatgtcaatacgcgaattcggacgactggcatctctaggaggaggattccttcttttatgacatgtttattttatatacattgatgctttccgacagtcggaagtaataaatgaatttatttcaagactacctatactcctttgacttgttcgactaatcttaccgcttactaaaatctcgaaatcacgcttgacctctcgcacgcaaatttttgctgctggacgctacgcactcggcccaattcttctcggtcctcgtcgtcgcaattgtcgttgcgttgatcttgcaccgaaggaatcagagaatagaatacc

SEQ ID NO: 85 - protein, 18 aa, artificial
  modified signal peptide B from human serum albumin
KWVTFISLLFLFSSSSRA

SEQ ID NO: 86 - DNA, 57 bp, artificial
  Codon-optimized DNA sequence coding for signal peptide ''E''
atgacccgactcacggtcctagcccttttggctggactgttggcgtcgtcccgcgca

SEQ ID NO: 87 - DNA, 57 bp, artificial
  Codon-optimized DNA sequence coding for signal peptide ''H5"
atggactggacctggcgattcttgtttgttgtcgccgcggctacgggagtgcaatcg

SEQ ID NO: 88 - DNA, 57 bp, artificial
  Codon-optimized DNA sequence coding for signal peptide ''H7"
atggagtttgggctgtcatgggtattcctcgttgccctgttccgaggtgtgcagtgc

SEQ ID NO: 89 - DNA, 66 bp, artificial
  Codon-optimized DNA sequence coding for signal peptide ''L1"
atggacatgcgagtcccggctcaacttctcggattactactgttgtggttgtcgggtgcccgctgc

SEQ ID NO: 90 - DNA, 54 bp, artificial
  Codon-optimized DNA sequence coding for signal peptide of the human BIP
atgaagctatccttggtcgcagccatgctgcttctcttgtcggctgcgcgagcc

SEQ ID NO: 91 - DNA, 51 bp, artificial
  Codon-optimized DNA sequence coding for signal peptide of the human PDI
atgctacgacgtgccttgctctgccttgcggtggctgccctggtccgcgca